European Patent Specification EP 3 710 484 B1, published October 25, 2023. Title: ANTIBODIES BINDING CTLA-4 AND USES THEREOF. Applicant: Harbour Biomed (Shanghai) Co., Ltd. The sequence listing filed with the application follows.

SEQUENCE LISTING (200 sequences)

SEQ ID NO: 1 - DNA, 1113 bp, Homo Sapiens
atggagaccgacaccctgctgctgtgggtgctgctgctgtgggtgcccggatccaccggctctgaggtgcagctggtggagattggaggaggcgagatccagccgggggggtccctgagactctcgtgtgcagcctctgggttcaacgtcagtaagaactacatgagttgggtccgccaggctccagggaaggggctggagtgggtctcagtaatctatagtggtggtggtacagaatacgcagcctccgtgaagggccgatttaacatctccagagacagttccaagaatatgttgtatcttcaaatgaacaacctgagagccgaggacacggccgtgtattattgtgcgagggccgtccccaggccccatgggactgatatctggggccaagggacaatggtcaccgtctcttcagagcccaaatcttgtgacaaaactcacacatgcccaccgtgcccagcacctgaactcctggggggaccgtcagtcttcctcttccccccaaaacccaaggacaccctcatgatctcccggacccctgaggtcacatgcgtggtggtggacgtgagccacgaagaccctgaggtcaagttcaactggtacgtggacggcgtggaggtgcataatgccaagacaaagccgcgggaggagcagtacaacagcacgtaccgggtggtcagcgtcctcaccgtcctgcaccaggactggctgaatggcaaggagtacaagtgcaaggtctccaacaaagccctcccagcccccatcgagaaaaccatctccaaagccaaagggcagccccgagaaccacaggtgtacaccctgcccccatcccgggaggagatgaccaagaaccaggtcagcctgacctgcctggtcaaaggcttctatcccagcgacatcgccgtggagtgggagagcaatgggcagccggagaacaactacaagaccacgcctcccgtgctggactccgacggctccttcttcctctacagcaagctcaccgtggacaagagcaggtggcagcaggggaacgtcttctcatgctccgtgatgcatgaggctctgcacaaccactacacgcagaagagcctctccctgtctccgggtaaa

SEQ ID NO: 2 - protein, 371 aa, Homo Sapiens
METDTLLLWVLLLWVPGSTGSEVQLVEIGGGEIQPGGSLRLSCAASGFNVSKNYMSWVRQAPGKGLEWVSVIYSGGGTEYAASVKGRFNISRDSSKNMLYLQMNNLRAEDTAVYYCARAVPRPHGTDIWGQGTMVTVSSEPKSCDKTHTCPPCPAPELLGGPSVFLFPPKPKDTLMISRTPEVTCVVVDVSHEDPEVKFNWYVDGVEVHNAKTKPREEQYNSTYRVVSVLTVLHQDWLNGKEYKCKVSNKALPAPIEKTISKAKGQPREPQVYTLPPSREEMTKNQVSLTCLVKGFYPSDIAVEWESNGQPENNYKTTPPVLDSDGSFFLYSKLTVDKSRWQQGNVFSCSVMHEALHNHYTQKSLSLSPGK

SEQ ID NO: 3 - protein, 118 aa, Homo Sapiens
EVQLVEIGGGEIQPGGSLRLSCAASGFNVSKNYMSWVRQAPGKGLEWVSVIYSGGGTEYAASVKGRFNISRDSSKNMLYLQMNNLRAEDTAVYYCARAVPRPHGTDIWGQGTMVTVSS

SEQ ID NO: 4 - protein, 10 aa, Homo Sapiens
GFNVSKNYMS

SEQ ID NO: 5 - protein, 16 aa, Homo Sapiens
VIYSGGGTEYAASVKG

SEQ ID NO: 6 - protein, 10 aa, Homo Sapiens
AVPRPHGTDI

SEQ ID NO: 7 - DNA, 1116 bp, Homo Sapiens
atggagaccgacaccctgctgctgtgggtgctgctgctgtgggtgcccggatccaccggctctgaggtgcagctggcggagactggaggaggcttgatccagcctggggggtccctgagactctcctgtgcagtctctgggttcaatgtcagtaagaattacatgagctgggtccgccaggttccagggaaggggctggagtgggtcgcagttgtttatagcggtggtagcaaaacctacgcagactccgtgaagggccgattcatcctctccagagacaattccgacaacacactgtatcttcaaatgaacaacctgagagccgaggacacggccgtgtattactgtgcgagagccgttcctcattcccccagttcttttgatatctggggccaagggacaatggtcaccgtctcttcagagcccaaatcttgtgacaaaactcacacatgcccaccgtgcccagcacctgaactcctggggggaccgtcagtcttcctcttccccccaaaacccaaggacaccctcatgatctcccggacccctgaggtcacatgcgtggtggtggacgtgagccacgaagaccctgaggtcaagttcaactggtacgtggacggcgtggaggtgcataatgccaagacaaagccgcgggaggagcagtacaacagcacgtaccgggtggtcagcgtcctcaccgtcctgcaccaggactggctgaatggcaaggagtacaagtgcaaggtctccaacaaagccctcccagcccccatcgagaaaaccatctccaaagccaaagggcagccccgagaaccacaggtgtacaccctgcccccatcccgggaggagatgaccaagaaccaggtcagcctgacctgcctggtcaaaggcttctatcccagcgacatcgccgtggagtgggagagcaatgggcagccggagaacaactacaagaccacgcctcccgtgctggactccgacggctccttcttcctctacagcaagctcaccgtggacaagagcaggtggcagcaggggaacgtcttctcatgctccgtgatgcatgaggctctgcacaaccactacacgcagaagagcctctccctgtctccgggtaaa

SEQ ID NO: 8 - protein, 372 aa, Homo Sapiens
METDTLLLWVLLLWVPGSTGSEVQLAETGGGLIQPGGSLRLSCAVSGFNVSKNYMSWVRQVPGKGLEWVAVVYSGGSKTYADSVKGRFILSRDNSDNTLYLQMNNLRAEDTAVYYCARAVPHSPSSFDIWGQGTMVTVSSEPKSCDKTHTCPPCPAPELLGGPSVFLFPPKPKDTLMISRTPEVTCVVVDVSHEDPEVKFNWYVDGVEVHNAKTKPREEQYNSTYRVVSVLTVLHQDWLNGKEYKCKVSNKALPAPIEKTISKAKGQPREPQVYTLPPSREEMTKNQVSLTCLVKGFYPSDIAVEWESNGQPENNYKTTPPVLDSDGSFFLYSKLTVDKSRWQQGNVFSCSVMHEALHNHYTQKSLSLSPGK

SEQ ID NO: 9 - protein, 119 aa, Homo Sapiens
EVQLAETGGGLIQPGGSLRLSCAVSGFNVSKNYMSWVRQVPGKGLEWVAVVYSGGSKTYADSVKGRFILSRDNSDNTLYLQMNNLRAEDTAVYYCARAVPHSPSSFDIWGQGTMVTVSS

SEQ ID NO: 10 - protein, 10 aa, Homo Sapiens
GFNVSKNYMS

SEQ ID NO: 11 - protein, 16 aa, Homo Sapiens)
VVYSGGSKTYADSVKG

SEQ ID NO: 12 - protein, 11 aa, Homo Sapiens
AVPHSPSSFDI

SEQ ID NO: 13 - DNA, 1116 bp, Homo Sapiens)
atggagaccgacaccctgctgctgtgggtgctgctgctgtgggtgcccggatccaccggctctgaggtgcagctggaggagactggaggagacttgatccagccgggggggtccctgagactctcctgtacagcctctgggtttaacgtcagtagaatctacatgagctgggtccgccaggctccagggaaggggctggagtgggtctcagtgatttatagcggtggaagtatatattacgcagattccgtgaggggccgatttaccatctccagagacagttccacgaacacggtgtttcttcaaatgaacagcctgagagccgaggactcggccgtgtattactgtgcgagagccgtcccaagtgcccctagttcttttgatatctggggccaagggacaatggtcaccgtctcttcagagcccaaatcttgtgacaaaactcacacatgcccaccgtgcccagcacctgaactcctggggggaccgtcagtcttcctcttccccccaaaacccaaggacaccctcatgatctcccggacccctgaggtcacatgcgtggtggtggacgtgagccacgaagaccctgaggtcaagttcaactggtacgtggacggcgtggaggtgcataatgccaagacaaagccgcgggaggagcagtacaacagcacgtaccgggtggtcagcgtcctcaccgtcctgcaccaggactggctgaatggcaaggagtacaagtgcaaggtctccaacaaagccctcccagcccccatcgagaaaaccatctccaaagccaaagggcagccccgagaaccacaggtgtacaccctgcccccatcccgggaggagatgaccaagaaccaggtcagcctgacctgcctggtcaaaggcttctatcccagcgacatcgccgtggagtgggagagcaatgggcagccggagaacaactacaagaccacgcctcccgtgctggactccgacggctccttcttcctctacagcaagctcaccgtggacaagagcaggtggcagcaggggaacgtcttctcatgctccgtgatgcatgaggctctgcacaaccactacacgcagaagagcctctccctgtctccgggtaaa

SEQ ID NO: 14 - protein, 372 aa, Homo Sapiens)
METDTLLLWVLLLWVPGSTGSEVQLEETGGDLIQPGGSLRLSCTASGFNVSRIYMSWVRQAPGKGLEWVSVIYSGGSIYYADSVRGRFTISRDSSTNTVFLQMNSLRAEDSAVYYCARAVPSAPSSFDIWGQGTMVTVSSEPKSCDKTHTCPPCPAPELLGGPSVFLFPPKPKDTLMISRTPEVTCVVVDVSHEDPEVKFNWYVDGVEVHNAKTKPREEQYNSTYRVVSVLTVLHQDWLNGKEYKCKVSNKALPAPIEKTISKAKGQPREPQVYTLPPSREEMTKNQVSLTCLVKGFYPSDIAVEWESNGQPENNYKTTPPVLDSDGSFFLYSKLTVDKSRWQQGNVFSCSVMHEALHNHYTQKSLSLSPGK

SEQ ID NO: 15 - protein, 119 aa, Homo Sapiens
EVQLEETGGDLIQPGGSLRLSCTASGFNVSRIYMSWVRQAPGKGLEWVSVIYSGGSIYYADSVRGRFTISRDSSTNTVFLQMNSLRAEDSAVYYCARAVPSAPSSFDIWGQGTMVTVSS

SEQ ID NO: 16 - protein, 10 aa, Homo Sapiens
GFNVSRIYMS

SEQ ID NO: 17 - protein, 16 aa, Homo Sapiens
VIYSGGSIYYADSVRG

SEQ ID NO: 18 - protein, 11 aa, Homo Sapiens
AVPSAPSSFDI

SEQ ID NO: 19 - DNA, 1119 bp, Homo Sapiens
atggagaccgacaccctgctgctgtgggtgctgctgctgtgggtgcccggatccaccggctctgaggtgcagctggtggagtccgggggaggcttagttcagcctggggggtccctgagactctcctgtgcagcctctggattcaccttcagtaactactggatgcactgggtccgccaagctccagggaaggggctggtgtgggtctcacgtattaatagtgatgggagtaacacaacctacgcggactccgtgaagggccgattcaccatctccagagacaacgccaagaacacgctgtatctgcaaatgaacagtctgagagccgaggacacggctgtgtattactgtgcaagatggttcggggagcactactacggaatggacgtctggggccaagggaccacggtcaccgtctcttcagagcccaaatcttgtgacaaaactcacacatgcccaccgtgcccagcacctgaactcctggggggaccgtcagtcttcctcttccccccaaaacccaaggacaccctcatgatctcccggacccctgaggtcacatgcgtggtggtggacgtgagccacgaagaccctgaggtcaagttcaactggtacgtggacggcgtggaggtgcataatgccaagacaaagccgcgggaggagcagtacaacagcacgtaccgggtggtcagcgtcctcaccgtcctgcaccaggactggctgaatggcaaggagtacaagtgcaaggtctccaacaaagccctcccagcccccatcgagaaaaccatctccaaagccaaagggcagccccgagaaccacaggtgtacaccctgcccccatcccgggaggagatgaccaagaaccaggtcagcctgacctgcctggtcaaaggcttctatcccagcgacatcgccgtggagtgggagagcaatgggcagccggagaacaactacaagaccacgcctcccgtgctggactccgacggctccttcttcctctacagcaagctcaccgtggacaagagcaggtggcagcaggggaacgtcttctcatgctccgtgatgcatgaggctctgcacaaccactacacgcagaagagcctctccctgtctccgggtaaa

SEQ ID NO: 20 - protein, 373 aa, Homo Sapiens
METDTLLLWVLLLWVPGSTGSEVQLVESGGGLVQPGGSLRLSCAASGFTFSNYWMHWVRQAPGKGLVWVSRINSDGSNTTYADSVKGRFTISRDNAKNTLYLQMNSLRAEDTAVYYCARWFGEHYYGMDVWGQGTTVTVSSEPKSCDKTHTCPPCPAPELLGGPSVFLFPPKPKDTLMISRTPEVTCVVVDVSHEDPEVKFNWYVDGVEVHNAKTKPREEQYNSTYRVVSVLTVLHQDWLNGKEYKCKVSNKALPAPIEKTISKAKGQPREPQVYTLPPSREEMTKNQVSLTCLVKGFYPSDIAVEWESNGQPENNYKTTPPVLDSDGSFFLYSKLTVDKSRWQQGNVFSCSVMHEALHNHYTQKSLSLSPGK

SEQ ID NO: 21 - protein, 120 aa, Homo Sapiens
EVQLVESGGGLVQPGGSLRLSCAASGFTFSNYWMHWVRQAPGKGLVWVSRINSDGSNTTYADSVKGRFTISRDNAKNTLYLQMNSLRAEDTAVYYCARWFGEHYYGMDVWGQGTTVTVSS

SEQ ID NO: 22 - protein, 10 aa, Homo Sapiens
GFTFSNYWMH

SEQ ID NO: 23 - protein, 17 aa, Homo Sapiens
RINSDGSNTTYADSVKG

SEQ ID NO: 24 - protein, 11 aa, Homo Sapiens
WFGEHYYGMDV

SEQ ID NO: 25 - DNA, 1116 bp, Homo Sapiens
atggagaccgacaccctgctgctgtgggtgctgctgctgtgggtgcccggatccaccggctctgaggtgcagctggtggagactggaggagggctgatccagccgggggggtccctgagactctcctgtgcagtctctgggttcaccgtcagaaacaactacatgagctgggcccgccaggttccagggaagggactggagtgggtctcagttatttatagcggtgggagtataacctacgcagactccgtgaagggccgattcatcatctccagagacaattccaacaacacgctatatcttcaaatgaacggtctgagagccgaggacacggccgtatattactgtgcgagagccgtcccacatgccccaagtgcttttgacatctggggccaggggacaatggtcaccgtctcttcagagcccaaatcttgtgacaaaactcacacatgcccaccgtgcccagcacctgaactcctggggggaccgtcagtcttcctcttccccccaaaacccaaggacaccctcatgatctcccggacccctgaggtcacatgcgtggtggtggacgtgagccacgaagaccctgaggtcaagttcaactggtacgtggacggcgtggaggtgcataatgccaagacaaagccgcgggaggagcagtacaacagcacgtaccgggtggtcagcgtcctcaccgtcctgcaccaggactggctgaatggcaaggagtacaagtgcaaggtctccaacaaagccctcccagcccccatcgagaaaaccatctccaaagccaaagggcagccccgagaaccacaggtgtacaccctgcccccatcccgggaggagatgaccaagaaccaggtcagcctgacctgcctggtcaaaggcttctatcccagcgacatcgccgtggagtgggagagcaatgggcagccggagaacaactacaagaccacgcctcccgtgctggactccgacggctccttcttcctctacagcaagctcaccgtggacaagagcaggtggcagcaggggaacgtcttctcatgctccgtgatgcatgaggctctgcacaaccactacacgcagaagagcctctccctgtctccgggtaaa

SEQ ID NO: 26 - protein, 372 aa, Homo Sapiens
METDTLLLWVLLLWVPGSTGSEVQLVETGGGLIQPGGSLRLSCAVSGFTVRNNYMSWARQVPGKGLEWVSVIYSGGSITYADSVKGRFIISRDNSNNTLYLQMNGLRAEDTAVYYCARAVPHAPSAFDIWGQGTMVTVSSEPKSCDKTHTCPPCPAPELLGGPSVFLFPPKPKDTLMISRTPEVTCVVVDVSHEDPEVKFNWYVDGVEVHNAKTKPREEQYNSTYRVVSVLTVLHQDWLNGKEYKCKVSNKALPAPIEKTISKAKGQPREPQVYTLPPSREEMTKNQVSLTCLVKGFYPSDIAVEWESNGQPENNYKTTPPVLDSDGSFFLYSKLTVDKSRWQQGNVFSCSVMHEALHNHYTQKSLSLSPGK

SEQ ID NO: 27 - protein, 119 aa, Homo Sapiens
EVQLVETGGGLIQPGGSLRLSCAVSGFTVRNNYMSWARQVPGKGLEWVSVIYSGGSITYADSVKGRFIISRDNSNNTLYLQMNGLRAEDTAVYYCARAVPHAPSAFDIWGQGTMVTVSS

SEQ ID NO: 28 - protein, 10 aa, Homo Sapiens
GFTVRNNYMS

SEQ ID NO: 29 - protein, 16 aa, Homo Sapiens
VIYSGGSITYADSVKG

SEQ ID NO: 30 - protein, 11 aa, Homo Sapiens
AVPHAPSAFDI

SEQ ID NO: 31 - DNA, 1113 bp, Homo Sapiens
atggagaccgacaccctgctgctgtgggtgctgctgctgtgggtgcccggatccaccggctctgaggtgcagctggtggagactggaggaggcttaatccagcctggggggtccctgagactctcctgtgcagcctctgggctcaatgtcagtaggcactacttaagctgggtccgccaggctccagggaaggggctggagtgggtcgcagtaatttatagcggtggtggtatagagtacgtagactccgtgaagggccgattcaccatctccagagacaatgccaacaacacgctgtatcttcaaatgagaagcctgagaaccgaagactcggccgtatattactgtgcgcgggccattcccagaccccatggttcggatatctggggccaagggacaatggtcaccgtctcttcagagcccaaatcttgtgacaaaactcacacatgcccaccgtgcccagcacctgaactcctggggggaccgtcagtcttcctcttccccccaaaacccaaggacaccctcatgatctcccggacccctgaggtcacatgcgtggtggtggacgtgagccacgaagaccctgaggtcaagttcaactggtacgtggacggcgtggaggtgcataatgccaagacaaagccgcgggaggagcagtacaacagcacgtaccgggtggtcagcgtcctcaccgtcctgcaccaggactggctgaatggcaaggagtacaagtgcaaggtctccaacaaagccctcccagcccccatcgagaaaaccatctccaaagccaaagggcagccccgagaaccacaggtgtacaccctgcccccatcccgggaggagatgaccaagaaccaggtcagcctgacctgcctggtcaaaggcttctatcccagcgacatcgccgtggagtgggagagcaatgggcagccggagaacaactacaagaccacgcctcccgtgctggactccgacggctccttcttcctctacagcaagctcaccgtggacaagagcaggtggcagcaggggaacgtcttctcatgctccgtgatgcatgaggctctgcacaaccactacacgcagaagagcctctccctgtctccgggtaaa

SEQ ID NO: 32 - protein, 371 aa, Homo Sapiens
METDTLLLWVLLLWVPGSTGSEVQLVETGGGLIQPGGSLRLSCAASGLNVSRHYLSWVRQAPGKGLEWVAVIYSGGGIEYVDSVKGRFTISRDNANNTLYLQMRSLRTEDSAVYYCARAIPRPHGSDIWGQGTMVTVSSEPKSCDKTHTCPPCPAPELLGGPSVFLFPPKPKDTLMISRTPEVTCVVVDVSHEDPEVKFNWYVDGVEVHNAKTKPREEQYNSTYRVVSVLTVLHQDWLNGKEYKCKVSNKALPAPIEKTISKAKGQPREPQVYTLPPSREEMTKNQVSLTCLVKGFYPSDIAVEWESNGQPENNYKTTPPVLDSDGSFFLYSKLTVDKSRWQQGNVFSCSVMHEALHNHYTQKSLSLSPGK

SEQ ID NO: 33 - protein, 118 aa, Homo Sapiens
EVQLVETGGGLIQPGGSLRLSCAASGLNVSRHYLSWVRQAPGKGLEWVAVIYSGGGIEYVDSVKGRFTISRDNANNTLYLQMRSLRTEDSAVYYCARAIPRPHGSDIWGQGTMVTVSS

SEQ ID NO: 34 - protein, 10 aa, Homo Sapiens
GLNVSRHYLS

SEQ ID NO: 35 - protein, 16 aa, Homo Sapiens
VIYSGGGIEYVDSVKG

SEQ ID NO: 36 - protein, 10 aa, Homo Sapiens
AIPRPHGSDI

SEQ ID NO: 37 - DNA, 1116 bp, Homo Sapiens
atggagaccgacaccctgctgctgtgggtgctgctgctgtgggtgcccggatccaccggctctgaggtgcagctggtggagactggaggaggcttgatccagcctggggggtccctgagactctcctgtgcagcctctgggttcaccgtcagtagcaactacatgagctgggtccgccaggctccagggaaggggctggagtgggtctcagttatttatagcggtggtagcacatactacgcagactccgtgaagggccgattcaccatctccagagacaattccaagaacacgctgtatcttcaaatgagcaacctgaccgccgaggacacggccgtgtattactgtgcgagagccgttccccactcccccagtgcttttgataggtggggccagggaaccctggtcaccgtctcttcagagcccaaatcttgtgacaaaactcacacatgcccaccgtgcccagcacctgaactcctggggggaccgtcagtcttcctcttccccccaaaacccaaggacaccctcatgatctcccggacccctgaggtcacatgcgtggtggtggacgtgagccacgaagaccctgaggtcaagttcaactggtacgtggacggcgtggaggtgcataatgccaagacaaagccgcgggaggagcagtacaacagcacgtaccgggtggtcagcgtcctcaccgtcctgcaccaggactggctgaatggcaaggagtacaagtgcaaggtctccaacaaagccctcccagcccccatcgagaaaaccatctccaaagccaaagggcagccccgagaaccacaggtgtacaccctgcccccatcccgggaggagatgaccaagaaccaggtcagcctgacctgcctggtcaaaggcttctatcccagcgacatcgccgtggagtgggagagcaatgggcagccggagaacaactacaagaccacgcctcccgtgctggactccgacggctccttcttcctctacagcaagctcaccgtggacaagagcaggtggcagcaggggaacgtcttctcatgctccgtgatgcatgaggctctgcacaaccactacacgcagaagagcctctccctgtctccgggtaaa

SEQ ID NO: 38 - protein, 372 aa, Homo Sapiens
METDTLLLWVLLLWVPGSTGSEVQLVETGGGLIQPGGSLRLSCAASGFTVSSNYMSWVRQAPGKGLEWVSVIYSGGSTYYADSVKGRFTISRDNSKNTLYLQMSNLTAEDTAVYYCARAVPHSPSAFDRWGQGTLVTVSSEPKSCDKTHTCPPCPAPELLGGPSVFLFPPKPKDTLMISRTPEVTCVVVDVSHEDPEVKFNWYVDGVEVHNAKTKPREEQYNSTYRVVSVLTVLHQDWLNGKEYKCKVSNKALPAPIEKTISKAKGQPREPQVYTLPPSREEMTKNQVSLTCLVKGFYPSDIAVEWESNGQPENNYKTTPPVLDSDGSFFLYSKLTVDKSRWQQGNVFSCSVMHEALHNHYTQKSLSLSPGK

SEQ ID NO: 39 - protein, 119 aa, Homo Sapiens
EVQLVETGGGLIQPGGSLRLSCAASGFTVSSNYMSWVRQAPGKGLEWVSVIYSGGSTYYADSVKGRFTISRDNSKNTLYLQMSNLTAEDTAVYYCARAVPHSPSAFDRWGQGTLVTVSS

SEQ ID NO: 40 - protein, 10 aa, Homo Sapiens
GFTVSSNYMS

SEQ ID NO: 41 - protein, 16 aa, Homo Sapiens
VIYSGGSTYYADSVKG

SEQ ID NO: 42 - protein, 11 aa, Homo Sapiens
AVPHSPSAFDR

SEQ ID NO: 43 - DNA, 1116 bp, Homo Sapiens
atggagaccgacaccctgctgctgtgggtgctgctgctgtgggtgcccggatccaccggctctgaggtgcagctggaggagactggaggagacttgatccagccgggggggtccctgagactctcctgtacagcctctgggtttaacgtcagtagaatctacatgagctgggtccgccaggctccagggaaggggctggagtgggtctcagtgatttatagcggtggaagtatatattacgcagattccgtgaggggccgatttaccatctccagagacagttccacgaacacggtgtatcttcaaatgaacagcctgagagccgaggactcggccgtgtattactgtgcgagagccgtcccacatgcccctagtaattttgataaatggggccaagggacaagggtcaccgtctcttcagagcccaaatcttgtgacaaaactcacacatgcccaccgtgcccagcacctgaactcctggggggaccgtcagtcttcctcttccccccaaaacccaaggacaccctcatgatctcccggacccctgaggtcacatgcgtggtggtggacgtgagccacgaagaccctgaggtcaagttcaactggtacgtggacggcgtggaggtgcataatgccaagacaaagccgcgggaggagcagtacaacagcacgtaccgggtggtcagcgtcctcaccgtcctgcaccaggactggctgaatggcaaggagtacaagtgcaaggtctccaacaaagccctcccagcccccatcgagaaaaccatctccaaagccaaagggcagccccgagaaccacaggtgtacaccctgcccccatcccgggaggagatgaccaagaaccaggtcagcctgacctgcctggtcaaaggcttctatcccagcgacatcgccgtggagtgggagagcaatgggcagccggagaacaactacaagaccacgcctcccgtgctggactccgacggctccttcttcctctacagcaagctcaccgtggacaagagcaggtggcagcaggggaacgtcttctcatgctccgtgatgcatgaggctctgcacaaccactacacgcagaagagcctctccctgtctccgggtaaa

SEQ ID NO: 44 - protein, 372 aa, Homo Sapiens
METDTLLLWVLLLWVPGSTGSEVQLEETGGDLIQPGGSLRLSCTASGFNVSRIYMSWVRQAPGKGLEWVSVIYSGGSIYYADSVRGRFTISRDSSTNTVYLQMNSLRAEDSAVYYCARAVPHAPSNFDKWGQGTRVTVSSEPKSCDKTHTCPPCPAPELLGGPSVFLFPPKPKDTLMISRTPEVTCVVVDVSHEDPEVKFNWYVDGVEVHNAKTKPREEQYNSTYRVVSVLTVLHQDWLNGKEYKCKVSNKALPAPIEKTISKAKGQPREPQVYTLPPSREEMTKNQVSLTCLVKGFYPSDIAVEWESNGQPENNYKTTPPVLDSDGSFFLYSKLTVDKSRWQQGNVFSCSVMHEALHNHYTQKSLSLSPGK

SEQ ID NO: 45 - protein, 119 aa, Homo Sapiens
EVQLEETGGDLIQPGGSLRLSCTASGFNVSRIYMSWVRQAPGKGLEWVSVIYSGGSIYYADSVRGRFTISRDSSTNTVYLQMNSLRAEDSAVYYCARAVPHAPSNFDKWGQGTRVTVSS

SEQ ID NO: 46 - protein, 10 aa, Homo Sapiens
GFNVSRIYMS

SEQ ID NO: 47 - protein, 16 aa, Homo Sapiens
VIYSGGSIYYADSVRG

SEQ ID NO: 48 - protein, 11 aa, Homo Sapiens
AVPHAPSNFDK

SEQ ID NO: 49 - DNA, 1125 bp, Homo Sapiens
atggagaccgacaccctgctgctgtgggtgctgctgctgtgggtgcccggatccaccggctctgaggtgcagctggtggagtctgggggaggcttggttcagccgggggggtccctgcgactctcctgtgtagcctctggattcaccttcagtaactattggatgcactgggtccgccaaattccagggaaggggatggtgtggatctcagaaattaacagtgacgggaataggacaggctatgcggactccgtaaagggccgattcaccatctccagagacaacgccaagaagatgttgtatctgcaaatgaacagtctgagagccgaggacacggctgtttattattgtgcaagaaactggggatcgggcccccatcataccgcttttgatggttggggccaagggacaatggtcaccgtctcttcagagcccaaatcttgtgacaaaactcacacatgcccaccgtgcccagcacctgaactcctggggggaccgtcagtcttcctcttccccccaaaacccaaggacaccctcatgatctcccggacccctgaggtcacatgcgtggtggtggacgtgagccacgaagaccctgaggtcaagttcaactggtacgtggacggcgtggaggtgcataatgccaagacaaagccgcgggaggagcagtacaacagcacgtaccgggtggtcagcgtcctcaccgtcctgcaccaggactggctgaatggcaaggagtacaagtgcaaggtctccaacaaagccctcccagcccccatcgagaaaaccatctccaaagccaaagggcagccccgagaaccacaggtgtacaccctgcccccatcccgggaggagatgaccaagaaccaggtcagcctgacctgcctggtcaaaggcttctatcccagcgacatcgccgtggagtgggagagcaatgggcagccggagaacaactacaagaccacgcctcccgtgctggactccgacggctccttcttcctctacagcaagctcaccgtggacaagagcaggtggcagcaggggaacgtcttctcatgctccgtgatgcatgaggctctgcacaaccactacacgcagaagagcctctccctgtctccgggtaaa

SEQ ID NO: 50 - protein, 375 aa, Homo Sapiens
METDTLLLWVLLLWVPGSTGSEVQLVESGGGLVQPGGSLRLSCVASGFTFSNYWMHWVRQIPGKGMVWISEINSDGNRTGYADSVKGRFTISRDNAKKMLYLQMNSLRAEDTAVYYCARNWGSGPHHTAFDGWGQGTMVTVSSEPKSCDKTHTCPPCPAPELLGGPSVFLFPPKPKDTLMISRTPEVTCVVVDVSHEDPEVKFNWYVDGVEVHNAKTKPREEQYNSTYRVVSVLTVLHQDWLNGKEYKCKVSNKALPAPIEKTISKAKGQPREPQVYTLPPSREEMTKNQVSLTCLVKGFYPSDIAVEWESNGQPENNYKTTPPVLDSDGSFFLYSKLTVDKSRWQQGNVFSCSVMHEALHNHYTQKSLSLSPGK

SEQ ID NO: 51 - protein, 122 aa, Homo Sapiens
EVQLVESGGGLVQPGGSLRLSCVASGFTFSNYWMHWVRQIPGKGMVWISEINSDGNRTGYADSVKGRFTISRDNAKKMLYLQMNSLRAEDTAVYYCARNWGSGPHHTAFDGWGQGTMVTVSS

SEQ ID NO: 52 - protein, 10 aa, Homo Sapiens
GFTFSNYWMH

SEQ ID NO: 53 - protein, 17 aa, Homo Sapiens
EINSDGNRTGYADSVKG

SEQ ID NO: 54 - protein, 13 aa, Homo Sapiens
NWGSGPHHTAFDG

SEQ ID NO: 55 - DNA, 1116 bp, Homo Sapiens
atggagaccgacaccctgctgctgtgggtgctgctgctgtgggtgcccggatccaccggctctgaggtgcagctggaggagactggaggagacttgatccagccgggggggtccctgagactctcctgtacagcctctgggtttaccgtcagtagaatctacatgagctgggtccgccaggctccagggaaggggctggagtgggtctcagtgatttatagcggtggaagtatatattacgcagattccgtgaggggccgatttaccatctccagagacagttccacgaacacggtgtttcttcaaatgaacagcctgagagccgaggactcggccgtgtattactgtgcgagagccgtcccaagtgcccctagttcttttgatatctggggccaagggacaatggtcaccgtctcttcagagcccaaatcttgtgacaaaactcacacatgcccaccgtgcccagcacctgaactcctggggggaccgtcagtcttcctcttccccccaaaacccaaggacaccctcatgatctcccggacccctgaggtcacatgcgtggtggtggacgtgagccacgaagaccctgaggtcaagttcaactggtacgtggacggcgtggaggtgcataatgccaagacaaagccgcgggaggagcagtacaacagcacgtaccgggtggtcagcgtcctcaccgtcctgcaccaggactggctgaatggcaaggagtacaagtgcaaggtctccaacaaagccctcccagcccccatcgagaaaaccatctccaaagccaaagggcagccccgagaaccacaggtgtacaccctgcccccatcccgggaggagatgaccaagaaccaggtcagcctgacctgcctggtcaaaggcttctatcccagcgacatcgccgtggagtgggagagcaatgggcagccggagaacaactacaagaccacgcctcccgtgctggactccgacggctccttcttcctctacagcaagctcaccgtggacaagagcaggtggcagcaggggaacgtcttctcatgctccgtgatgcatgaggctctgcacaaccactacacgcagaagagcctctccctgtctccgggtaaa

SEQ ID NO: 56 - protein, 372 aa, Homo Sapiens
METDTLLLWVLLLWVPGSTGSEVQLEETGGDLIQPGGSLRLSCTASGFTVSRIYMSWVRQAPGKGLEWVSVIYSGGSIYYADSVRGRFTISRDSSTNTVFLQMNSLRAEDSAVYYCARAVPSAPSSFDIWGQGTMVTVSSEPKSCDKTHTCPPCPAPELLGGPSVFLFPPKPKDTLMISRTPEVTCVVVDVSHEDPEVKFNWYVDGVEVHNAKTKPREEQYNSTYRVVSVLTVLHQDWLNGKEYKCKVSNKALPAPIEKTISKAKGQPREPQVYTLPPSREEMTKNQVSLTCLVKGFYPSDIAVEWESNGQPENNYKTTPPVLDSDGSFFLYSKLTVDKSRWQQGNVFSCSVMHEALHNHYTQKSLSLSPGK

SEQ ID NO: 57 - protein, 119 aa, Homo Sapiens
EVQLEETGGDLIQPGGSLRLSCTASGFTVSRIYMSWVRQAPGKGLEWVSVIYSGGSIYYADSVRGRFTISRDSSTNTVFLQMNSLRAEDSAVYYCARAVPSAPSSFDIWGQGTMVTVSS

SEQ ID NO: 58 - protein, 10 aa, Homo Sapiens
GFTVSRIYMS

SEQ ID NO: 59 - protein, 16 aa, Homo Sapiens
VIYSGGSIYYADSVRG

SEQ ID NO: 60 - protein, 11 aa, Homo Sapiens
AVPSAPSSFDI

SEQ ID NO: 61 - DNA, 1116 bp, Homo Sapiens
atggagaccgacaccctgctgctgtgggtgctgctgctgtgggtgcccggatccaccggctctgaggtgcagctggtggagagcggaggaggcttgatccagccgggggggtccctgagactctcctgtgccgcctctgggtttaccgtcagtagaatctacatgagctgggtccgccaggctccagggaaggggctggagtgggtctcagtgatttatagcggtggaagtatatattacgcagattccgtgaagggccgatttaccatctccagagacagttccaagaacacggtgtaccttcaaatgaacagcctgagagccgaggacaccgccgtgtattactgtgcgagagccgtcccaagtgcccctagttcttttgatatctggggccaagggacaatggtcaccgtctcttcagagcccaaatcttgtgacaaaactcacacatgcccaccgtgcccagcacctgaactcctggggggaccgtcagtcttcctcttccccccaaaacccaaggacaccctcatgatctcccggacccctgaggtcacatgcgtggtggtggacgtgagccacgaagaccctgaggtcaagttcaactggtacgtggacggcgtggaggtgcataatgccaagacaaagccgcgggaggagcagtacaacagcacgtaccgggtggtcagcgtcctcaccgtcctgcaccaggactggctgaatggcaaggagtacaagtgcaaggtctccaacaaagccctcccagcccccatcgagaaaaccatctccaaagccaaagggcagccccgagaaccacaggtgtacaccctgcccccatcccgggaggagatgaccaagaaccaggtcagcctgacctgcctggtcaaaggcttctatcccagcgacatcgccgtggagtgggagagcaatgggcagccggagaacaactacaagaccacgcctcccgtgctggactccgacggctccttcttcctctacagcaagctcaccgtggacaagagcaggtggcagcaggggaacgtcttctcatgctccgtgatgcatgaggctctgcacaaccactacacgcagaagagcctctccctgtctccgggtaaa

SEQ ID NO: 62 - protein, 372 aa, Homo Sapiens
METDTLLLWVLLLWVPGSTGSEVQLVESGGGLIQPGGSLRLSCAASGFTVSRIYMSWVRQAPGKGLEWVSVIYSGGSIYYADSVKGRFTISRDSSKNTVYLQMNSLRAEDTAVYYCARAVPSAPSSFDIWGQGTMVTVSSEPKSCDKTHTCPPCPAPELLGGPSVFLFPPKPKDTLMISRTPEVTCVVVDVSHEDPEVKFNWYVDGVEVHNAKTKPREEQYNSTYRVVSVLTVLHQDWLNGKEYKCKVSNKALPAPIEKTISKAKGQPREPQVYTLPPSREEMTKNQVSLTCLVKGFYPSDIAVEWESNGQPENNYKTTPPVLDSDGSFFLYSKLTVDKSRWQQGNVFSCSVMHEALHNHYTQKSLSLSPGK

SEQ ID NO: 63 - protein, 119 aa, Homo Sapiens
EVQLVESGGGLIQPGGSLRLSCAASGFTVSRIYMSWVRQAPGKGLEWVSVIYSGGSIYYADSVKGRFTISRDSSKNTVYLQMNSLRAEDTAVYYCARAVPSAPSSFDIWGQGTMVTVSS

SEQ ID NO: 64 - protein, 10 aa, Homo Sapiens
GFTVSRIYMS

SEQ ID NO: 65 - protein, 16 aa, Homo Sapiens
VIYSGGSIYYADSVKG

SEQ ID NO: 66 - protein, 11 aa, Homo Sapiens
AVPSAPSSFDI

SEQ ID NO: 67 - DNA, 1116 bp, Homo Sapiens
atggagaccgacaccctgctgctgtgggtgctgctgctgtgggtgcccggatccaccggctctgaggtgcagctggtggagactggaggagggctgatccagccgggggggtccctgagactctcctgtgcagtctctgggttcaccgtcagaaacaactacatgagctgggcccgccaggttccagggaagggactggagtgggtctcagttatttatagcggtgggagtataacctacgcagactccgtgaagggccgattcatcatctccagagacaattccaagaacacgctatatcttcaaatgaacggtctgagagccgaggacacggccgtatattactgtgcgagagccgtcccacatgccccaagtgcttttgacatctggggccaggggacaatggtcaccgtctcttcagagcccaaatcttgtgacaaaactcacacatgcccaccgtgcccagcacctgaactcctggggggaccgtcagtcttcctcttccccccaaaacccaaggacaccctcatgatctcccggacccctgaggtcacatgcgtggtggtggacgtgagccacgaagaccctgaggtcaagttcaactggtacgtggacggcgtggaggtgcataatgccaagacaaagccgcgggaggagcagtacaacagcacgtaccgggtggtcagcgtcctcaccgtcctgcaccaggactggctgaatggcaaggagtacaagtgcaaggtctccaacaaagccctcccagcccccatcgagaaaaccatctccaaagccaaagggcagccccgagaaccacaggtgtacaccctgcccccatcccgggaggagatgaccaagaaccaggtcagcctgacctgcctggtcaaaggcttctatcccagcgacatcgccgtggagtgggagagcaatgggcagccggagaacaactacaagaccacgcctcccgtgctggactccgacggctccttcttcctctacagcaagctcaccgtggacaagagcaggtggcagcaggggaacgtcttctcatgctccgtgatgcatgaggctctgcacaaccactacacgcagaagagcctctccctgtctccgggtaaa

SEQ ID NO: 68 - protein, 372 aa, Homo Sapiens
METDTLLLWVLLLWVPGSTGSEVQLVETGGGLIQPGGSLRLSCAVSGFTVRNNYMSWARQVPGKGLEWVSVIYSGGSITYADSVKGRFIISRDNSKNTLYLQMNGLRAEDTAVYYCARAVPHAPSAFDIWGQGTMVTVSSEPKSCDKTHTCPPCPAPELLGGPSVFLFPPKPKDTLMISRTPEVTCVVVDVSHEDPEVKFNWYVDGVEVHNAKTKPREEQYNSTYRVVSVLTVLHQDWLNGKEYKCKVSNKALPAPIEKTISKAKGQPREPQVYTLPPSREEMTKNQVSLTCLVKGFYPSDIAVEWESNGQPENNYKTTPPVLDSDGSFFLYSKLTVDKSRWQQGNVFSCSVMHEALHNHYTQKSLSLSPGK

SEQ ID NO: 69 - protein, 119 aa, Homo Sapiens
EVQLVETGGGLIQPGGSLRLSCAVSGFTVRNNYMSWARQVPGKGLEWVSVIYSGGSITYADSVKGRFIISRDNSKNTLYLQMNGLRAEDTAVYYCARAVPHAPSAFDIWGQGTMVTVSS

SEQ ID NO: 70 - protein, 10 aa, Homo Sapiens
GFTVRNNYMS

SEQ ID NO: 71 - protein, 16 aa, Homo Sapiens
VIYSGGSITYADSVKG

SEQ ID NO: 72 - protein, 11 aa, Homo Sapiens
AVPHAPSAFDI

SEQ ID NO: 73 - DNA, 1116 bp, Homo Sapiens
atggagaccgacaccctgctgctgtgggtgctgctgctgtgggtgcccggatccaccggctctgaggtgcagctggtggagagcggaggagggctgatccagccgggggggtccctgagactctcctgtgcagcctctgggttcaccgtcagaaacaactacatgagctgggtgcgccaggccccagggaagggactggagtgggtctcagttatttatagcggtgggagtataacctacgcagactccgtgaagggccgattcaccatctccagagacaattccaagaacacgctatatcttcaaatgaacagcctgagagccgaggacacggccgtatattactgtgcgagagccgtcccacatgccccaagtgcttttgacatctggggccaggggacaatggtcaccgtctcttcagagcccaaatcttgtgacaaaactcacacatgcccaccgtgcccagcacctgaactcctggggggaccgtcagtcttcctcttccccccaaaacccaaggacaccctcatgatctcccggacccctgaggtcacatgcgtggtggtggacgtgagccacgaagaccctgaggtcaagttcaactggtacgtggacggcgtggaggtgcataatgccaagacaaagccgcgggaggagcagtacaacagcacgtaccgggtggtcagcgtcctcaccgtcctgcaccaggactggctgaatggcaaggagtacaagtgcaaggtctccaacaaagccctcccagcccccatcgagaaaaccatctccaaagccaaagggcagccccgagaaccacaggtgtacaccctgcccccatcccgggaggagatgaccaagaaccaggtcagcctgacctgcctggtcaaaggcttctatcccagcgacatcgccgtggagtgggagagcaatgggcagccggagaacaactacaagaccacgcctcccgtgctggactccgacggctccttcttcctctacagcaagctcaccgtggacaagagcaggtggcagcaggggaacgtcttctcatgctccgtgatgcatgaggctctgcacaaccactacacgcagaagagcctctccctgtctccgggtaaa

SEQ ID NO: 74 - protein, 372 aa, Homo Sapiens
METDTLLLWVLLLWVPGSTGSEVQLVESGGGLIQPGGSLRLSCAASGFTVRNNYMSWVRQAPGKGLEWVSVIYSGGSITYADSVKGRFTISRDNSKNTLYLQMNSLRAEDTAVYYCARAVPHAPSAFDIWGQGTMVTVSSEPKSCDKTHTCPPCPAPELLGGPSVFLFPPKPKDTLMISRTPEVTCVVVDVSHEDPEVKFNWYVDGVEVHNAKTKPREEQYNSTYRVVSVLTVLHQDWLNGKEYKCKVSNKALPAPIEKTISKAKGQPREPQVYTLPPSREEMTKNQVSLTCLVKGFYPSDIAVEWESNGQPENNYKTTPPVLDSDGSFFLYSKLTVDKSRWQQGNVFSCSVMHEALHNHYTQKSLSLSPGK

SEQ ID NO: 75 - protein, 119 aa, Homo Sapiens
EVQLVESGGGLIQPGGSLRLSCAASGFTVRNNYMSWVRQAPGKGLEWVSVIYSGGSITYADSVKGRFTISRDNSKNTLYLQMNSLRAEDTAVYYCARAVPHAPSAFDIWGQGTMVTVSS

SEQ ID NO: 76 - protein, 10 aa, Homo Sapiens
GFTVRNNYMS

SEQ ID NO: 77 - protein, 16 aa, Homo Sapiens
VIYSGGSITYADSVKG

SEQ ID NO: 78 - protein, 11 aa, Homo Sapiens
AVPHAPSAFDI

SEQ ID NO: 79 - DNA, 1116 bp, Homo Sapiens
atggagaccgacaccctgctgctgtgggtgctgctgctgtgggtgcccggatccaccggctctgaggtgcagctggtggagactggaggaggcttgatccagcctggggggtccctgagactctcctgtgcagcctctgggttcaccgtcagtagcaactacatgagctgggtccgccaggctccagggaaggggctggagtgggtctcagttatttatagcggtggtagcacatactacgcagactccgtgaagggccgattcaccatctccagagacaattccaagaacacgctgtatcttcaaatgagcagcctgagggccgaggacacggccgtgtattactgtgcgagagccgttccccactcccccagtgcttttgataggtggggccagggaaccctggtcaccgtctcttcagagcccaaatcttgtgacaaaactcacacatgcccaccgtgcccagcacctgaactcctggggggaccgtcagtcttcctcttccccccaaaacccaaggacaccctcatgatctcccggacccctgaggtcacatgcgtggtggtggacgtgagccacgaagaccctgaggtcaagttcaactggtacgtggacggcgtggaggtgcataatgccaagacaaagccgcgggaggagcagtacaacagcacgtaccgggtggtcagcgtcctcaccgtcctgcaccaggactggctgaatggcaaggagtacaagtgcaaggtctccaacaaagccctcccagcccccatcgagaaaaccatctccaaagccaaagggcagccccgagaaccacaggtgtacaccctgcccccatcccgggaggagatgaccaagaaccaggtcagcctgacctgcctggtcaaaggcttctatcccagcgacatcgccgtggagtgggagagcaatgggcagccggagaacaactacaagaccacgcctcccgtgctggactccgacggctccttcttcctctacagcaagctcaccgtggacaagagcaggtggcagcaggggaacgtcttctcatgctccgtgatgcatgaggctctgcacaaccactacacgcagaagagcctctccctgtctccgggtaaa

SEQ ID NO: 80 - protein, 372 aa, Homo Sapiens
METDTLLLWVLLLWVPGSTGSEVQLVETGGGLIQPGGSLRLSCAASGFTVSSNYMSWVRQAPGKGLEWVSVIYSGGSTYYADSVKGRFTISRDNSKNTLYLQMSSLRAEDTAVYYCARAVPHSPSAFDRWGQGTLVTVSSEPKSCDKTHTCPPCPAPELLGGPSVFLFPPKPKDTLMISRTPEVTCVVVDVSHEDPEVKFNWYVDGVEVHNAKTKPREEQYNSTYRVVSVLTVLHQDWLNGKEYKCKVSNKALPAPIEKTISKAKGQPREPQVYTLPPSREEMTKNQVSLTCLVKGFYPSDIAVEWESNGQPENNYKTTPPVLDSDGSFFLYSKLTVDKSRWQQGNVFSCSVMHEALHNHYTQKSLSLSPGK

SEQ ID NO: 81 - protein, 119 aa, Homo Sapiens
EVQLVETGGGLIQPGGSLRLSCAASGFTVSSNYMSWVRQAPGKGLEWVSVIYSGGSTYYADSVKGRFTISRDNSKNTLYLQMSSLRAEDTAVYYCARAVPHSPSAFDRWGQGTLVTVSS

SEQ ID NO: 82 - protein, 10 aa, Homo Sapiens
GFTVSSNYMS

SEQ ID NO: 83 - protein, 16 aa, Homo Sapiens
VIYSGGSTYYADSVKG

SEQ ID NO: 84 - protein, 11 aa, Homo Sapiens
AVPHSPSAFDR

SEQ ID NO: 85 - DNA, 1116 bp, Homo Sapiens
atggagaccgacaccctgctgctgtgggtgctgctgctgtgggtgcccggatccaccggctctgaggtgcagctggtggagagcggaggaggcttgatccagcctggggggtccctgagactctcctgtgcagcctctgggttcaccgtcagtagcaactacatgagctgggtccgccaggctccagggaaggggctggagtgggtctcagttatttatagcggtggtagcacatactacgcagactccgtgaagggccgattcaccatctccagagacaattccaagaacacgctgtatcttcaaatgaacagcctgagggccgaggacacggccgtgtattactgtgcgagagccgttccccactcccccagtgcttttgataggtggggccagggaaccctggtcaccgtctcttcagagcccaaatcttgtgacaaaactcacacatgcccaccgtgcccagcacctgaactcctggggggaccgtcagtcttcctcttccccccaaaacccaaggacaccctcatgatctcccggacccctgaggtcacatgcgtggtggtggacgtgagccacgaagaccctgaggtcaagttcaactggtacgtggacggcgtggaggtgcataatgccaagacaaagccgcgggaggagcagtacaacagcacgtaccgggtggtcagcgtcctcaccgtcctgcaccaggactggctgaatggcaaggagtacaagtgcaaggtctccaacaaagccctcccagcccccatcgagaaaaccatctccaaagccaaagggcagccccgagaaccacaggtgtacaccctgcccccatcccgggaggagatgaccaagaaccaggtcagcctgacctgcctggtcaaaggcttctatcccagcgacatcgccgtggagtgggagagcaatgggcagccggagaacaactacaagaccacgcctcccgtgctggactccgacggctccttcttcctctacagcaagctcaccgtggacaagagcaggtggcagcaggggaacgtcttctcatgctccgtgatgcatgaggctctgcacaaccactacacgcagaagagcctctccctgtctccgggtaaa

SEQ ID NO: 86 - protein, 372 aa, Homo Sapiens
METDTLLLWVLLLWVPGSTGSEVQLVESGGGLIQPGGSLRLSCAASGFTVSSNYMSWVRQAPGKGLEWVSVIYSGGSTYYADSVKGRFTISRDNSKNTLYLQMNSLRAEDTAVYYCARAVPHSPSAFDRWGQGTLVTVSSEPKSCDKTHTCPPCPAPELLGGPSVFLFPPKPKDTLMISRTPEVTCVVVDVSHEDPEVKFNWYVDGVEVHNAKTKPREEQYNSTYRVVSVLTVLHQDWLNGKEYKCKVSNKALPAPIEKTISKAKGQPREPQVYTLPPSREEMTKNQVSLTCLVKGFYPSDIAVEWESNGQPENNYKTTPPVLDSDGSFFLYSKLTVDKSRWQQGNVFSCSVMHEALHNHYTQKSLSLSPGK

SEQ ID NO: 87 - protein, 119 aa, Homo Sapiens
EVQLVESGGGLIQPGGSLRLSCAASGFTVSSNYMSWVRQAPGKGLEWVSVIYSGGSTYYADSVKGRFTISRDNSKNTLYLQMNSLRAEDTAVYYCARAVPHSPSAFDRWGQGTLVTVSS

SEQ ID NO: 88 - protein, 10 aa, Homo Sapiens
GFTVSSNYMS

SEQ ID NO: 89 - protein, 16 aa, Homo Sapiens
VIYSGGSTYYADSVKG

SEQ ID NO: 90 - protein, 11 aa, Homo Sapiens
AVPHSPSAFDR

SEQ ID NO: 91 - DNA, 1116 bp, Homo Sapiens
atggagaccgacaccctgctgctgtgggtgctgctgctgtgggtgcccggatccaccggctctgaggtgcagctggaggagactggaggagacttgatccagccgggggggtccctgagactctcctgtacagcctctgggtttaccgtcagtagaatctacatgagctgggtccgccaggctccagggaaggggctggagtgggtctcagtgatttatagcggtggaagtatatattacgcagattccgtgaggggccgatttaccatctccagagacagttccacgaacacggtgtatcttcaaatgaacagcctgagagccgaggactcggccgtgtattactgtgcgagagccgtcccacatgcccctagtaattttgataaatggggccaagggacaagggtcaccgtctcttcagagcccaaatcttgtgacaaaactcacacatgcccaccgtgcccagcacctgaactcctggggggaccgtcagtcttcctcttccccccaaaacccaaggacaccctcatgatctcccggacccctgaggtcacatgcgtggtggtggacgtgagccacgaagaccctgaggtcaagttcaactggtacgtggacggcgtggaggtgcataatgccaagacaaagccgcgggaggagcagtacaacagcacgtaccgggtggtcagcgtcctcaccgtcctgcaccaggactggctgaatggcaaggagtacaagtgcaaggtctccaacaaagccctcccagcccccatcgagaaaaccatctccaaagccaaagggcagccccgagaaccacaggtgtacaccctgcccccatcccgggaggagatgaccaagaaccaggtcagcctgacctgcctggtcaaaggcttctatcccagcgacatcgccgtggagtgggagagcaatgggcagccggagaacaactacaagaccacgcctcccgtgctggactccgacggctccttcttcctctacagcaagctcaccgtggacaagagcaggtggcagcaggggaacgtcttctcatgctccgtgatgcatgaggctctgcacaaccactacacgcagaagagcctctccctgtctccgggtaaa

SEQ ID NO: 92 - protein, 372 aa, Homo Sapiens
METDTLLLWVLLLWVPGSTGSEVQLEETGGDLIQPGGSLRLSCTASGFTVSRIYMSWVRQAPGKGLEWVSVIYSGGSIYYADSVRGRFTISRDSSTNTVYLQMNSLRAEDSAVYYCARAVPHAPSNFDKWGQGTRVTVSSEPKSCDKTHTCPPCPAPELLGGPSVFLFPPKPKDTLMISRTPEVTCVVVDVSHEDPEVKFNWYVDGVEVHNAKTKPREEQYNSTYRVVSVLTVLHQDWLNGKEYKCKVSNKALPAPIEKTISKAKGQPREPQVYTLPPSREEMTKNQVSLTCLVKGFYPSDIAVEWESNGQPENNYKTTPPVLDSDGSFFLYSKLTVDKSRWQQGNVFSCSVMHEALHNHYTQKSLSLSPGK

SEQ ID NO: 93 - protein, 119 aa, Homo Sapiens
EVQLEETGGDLIQPGGSLRLSCTASGFTVSRIYMSWVRQAPGKGLEWVSVIYSGGSIYYADSVRGRFTISRDSSTNTVYLQMNSLRAEDSAVYYCARAVPHAPSNFDKWGQGTRVTVSS

SEQ ID NO: 94 - protein, 10 aa, Homo Sapiens
GFTVSRIYMS

SEQ ID NO: 95 - protein, 16 aa, Homo Sapiens
VIYSGGSIYYADSVRG

SEQ ID NO: 96 - protein, 11 aa, Homo Sapiens
AVPHAPSNFDK

SEQ ID NO: 97 - DNA, 1116 bp, Homo Sapiens
atggagaccgacaccctgctgctgtgggtgctgctgctgtgggtgcccggatccaccggctctgaggtgcagctggcggagactggaggaggcttgatccagcctggggggtccctgagactctcctgtgcagtctctgggttcaccgtcagtaagaattacatgagctgggtccgccaggttccagggaaggggctggagtgggtcgcagttgtttatagcggtggtagcaaaacctacgcagactccgtgaagggccgattcatcctctccagagacaattccgacaacacactgtatcttcaaatgaacaacctgagagccgaggacacggccgtgtattactgtgcgagagccgttcctcattcccccagttcttttgatatctggggccaagggacaatggtcaccgtctcttcagagcccaaatcttgtgacaaaactcacacatgcccaccgtgcccagcacctgaactcctggggggaccgtcagtcttcctcttccccccaaaacccaaggacaccctcatgatctcccggacccctgaggtcacatgcgtggtggtggacgtgagccacgaagaccctgaggtcaagttcaactggtacgtggacggcgtggaggtgcataatgccaagacaaagccgcgggaggagcagtacaacagcacgtaccgggtggtcagcgtcctcaccgtcctgcaccaggactggctgaatggcaaggagtacaagtgcaaggtctccaacaaagccctcccagcccccatcgagaaaaccatctccaaagccaaagggcagccccgagaaccacaggtgtacaccctgcccccatcccgggaggagatgaccaagaaccaggtcagcctgacctgcctggtcaaaggcttctatcccagcgacatcgccgtggagtgggagagcaatgggcagccggagaacaactacaagaccacgcctcccgtgctggactccgacggctccttcttcctctacagcaagctcaccgtggacaagagcaggtggcagcaggggaacgtcttctcatgctccgtgatgcatgaggctctgcacaaccactacacgcagaagagcctctccctgtctccgggtaaa

SEQ ID NO: 98 - protein, 372 aa, Homo Sapiens
METDTLLLWVLLLWVPGSTGSEVQLVESGGGLIQPGGSLRLSCAASGFTVSRIYMSWVRQAPGKGLEWVSVIYSGGSIYYADSVKGRFTISRDSSKNTVYLQMNSLRAEDTAVYYCARAVPHAPSNFDKWGQGTLVTVSSEPKSCDKTHTCPPCPAPELLGGPSVFLFPPKPKDTLMISRTPEVTCVVVDVSHEDPEVKFNWYVDGVEVHNAKTKPREEQYNSTYRVVSVLTVLHQDWLNGKEYKCKVSNKALPAPIEKTISKAKGQPREPQVYTLPPSREEMTKNQVSLTCLVKGFYPSDIAVEWESNGQPENNYKTTPPVLDSDGSFFLYSKLTVDKSRWQQGNVFSCSVMHEALHNHYTQKSLSLSPGK

SEQ ID NO: 99 - protein, 119 aa, Homo Sapiens
EVQLVESGGGLIQPGGSLRLSCAASGFTVSRIYMSWVRQAPGKGLEWVSVIYSGGSIYYADSVKGRFTISRDSSKNTVYLQMNSLRAEDTAVYYCARAVPHAPSNFDKWGQGTLVTVSS

SEQ ID NO: 100 - protein, 10 aa, Homo Sapiens
GFTVSRIYMS

SEQ ID NO: 101 - protein, 16 aa, Homo Sapiens
VIYSGGSIYYADSVKG

SEQ ID NO: 102 - protein, 11 aa, Homo Sapiens
AVPHAPSNFDK

SEQ ID NO: 103 - DNA, 1116 bp, Homo Sapiens; identical to SEQ ID NO: 97

SEQ ID NO: 104 - protein, 372 aa, Homo Sapiens
METDTLLLWVLLLWVPGSTGSEVQLAETGGGLIQPGGSLRLSCAVSGFTVSKNYMSWVRQVPGKGLEWVAVVYSGGSKTYADSVKGRFILSRDNSDNTLYLQMNNLRAEDTAVYYCARAVPHSPSSFDIWGQGTMVTVSSEPKSCDKTHTCPPCPAPELLGGPSVFLFPPKPKDTLMISRTPEVTCVVVDVSHEDPEVKFNWYVDGVEVHNAKTKPREEQYNSTYRVVSVLTVLHQDWLNGKEYKCKVSNKALPAPIEKTISKAKGQPREPQVYTLPPSREEMTKNQVSLTCLVKGFYPSDIAVEWESNGQPENNYKTTPPVLDSDGSFFLYSKLTVDKSRWQQGNVFSCSVMHEALHNHYTQKSLSLSPGK

SEQ ID NO: 105 - protein, 119 aa, Homo Sapiens
EVQLAETGGGLIQPGGSLRLSCAVSGFTVSKNYMSWVRQVPGKGLEWVAVVYSGGSKTYADSVKGRFILSRDNSDNTLYLQMNNLRAEDTAVYYCARAVPHSPSSFDIWGQGTMVTVSS

SEQ ID NO: 106 - protein, 10 aa, Homo Sapiens
GFTVSKNYMS

SEQ ID NO: 107 - protein, 16 aa, Homo Sapiens
VVYSGGSKTYADSVKG

SEQ ID NO: 108 - protein, 11 aa, Homo Sapiens
AVPHSPSSFDI

SEQ ID NO: 109 - DNA, 1116 bp, Homo Sapiens
atggagaccgacaccctgctgctgtgggtgctgctgctgtgggtgcccggatccaccggctctgaggtgcagctggtggagagcggaggaggcttgatccagcctggggggtccctgagactctcctgtgcagtctctgggttcaccgtcagtaagaattacatgagctgggtccgccaggccccagggaaggggctggagtgggtcagcgttgtttatagcggtggtagcaaaacctacgcagactccgtgaagggccgattcaccatctccagagacaattccaagaacacactgtatcttcaaatgaacagcctgagagccgaggacacggccgtgtattactgtgcgagagccgttcctcattcccccagttcttttgatatctggggccaagggacaatggtcaccgtctcttcagagcccaaatcttgtgacaaaactcacacatgcccaccgtgcccagcacctgaactcctggggggaccgtcagtcttcctcttccccccaaaacccaaggacaccctcatgatctcccggacccctgaggtcacatgcgtggtggtggacgtgagccacgaagaccctgaggtcaagttcaactggtacgtggacggcgtggaggtgcataatgccaagacaaagccgcgggaggagcagtacaacagcacgtaccgggtggtcagcgtcctcaccgtcctgcaccaggactggctgaatggcaaggagtacaagtgcaaggtctccaacaaagccctcccagcccccatcgagaaaaccatctccaaagccaaagggcagccccgagaaccacaggtgtacaccctgcccccatcccgggaggagatgaccaagaaccaggtcagcctgacctgcctggtcaaaggcttctatcccagcgacatcgccgtggagtgggagagcaatgggcagccggagaacaactacaagaccacgcctcccgtgctggactccgacggctccttcttcctctacagcaagctcaccgtggacaagagcaggtggcagcaggggaacgtcttctcatgctccgtgatgcatgaggctctgcacaaccactacacgcagaagagcctctccctgtctccgggtaaa

SEQ ID NO: 110 - protein, 372 aa, Homo Sapiens
METDTLLLWVLLLWVPGSTGSEVQLVESGGGLIQPGGSLRLSCAVSGFTVSKNYMSWVRQAPGKGLEWVSVVYSGGSKTYADSVKGRFTISRDNSKNTLYLQMNSLRAEDTAVYYCARAVPHSPSSFDIWGQGTMVTVSSEPKSCDKTHTCPPCPAPELLGGPSVFLFPPKPKDTLMISRTPEVTCVVVDVSHEDPEVKFNWYVDGVEVHNAKTKPREEQYNSTYRVVSVLTVLHQDWLNGKEYKCKVSNKALPAPIEKTISKAKGQPREPQVYTLPPSREEMTKNQVSLTCLVKGFYPSDIAVEWESNGQPENNYKTTPPVLDSDGSFFLYSKLTVDKSRWQQGNVFSCSVMHEALHNHYTQKSLSLSPGK

SEQ ID NO: 111 - protein, 119 aa, Homo Sapiens
EVQLVESGGGLIQPGGSLRLSCAVSGFTVSKNYMSWVRQAPGKGLEWVSVVYSGGSKTYADSVKGRFTISRDNSKNTLYLQMNSLRAEDTAVYYCARAVPHSPSSFDIWGQGTMVTVSS

SEQ ID NO: 112 - protein, 10 aa, Homo Sapiens
GFTVSKNYMS

SEQ ID NO: 113 - protein, 16 aa, Homo Sapiens
VVYSGGSKTYADSVKG

SEQ ID NO: 114 - protein, 11 aa, Homo Sapiens
AVPHSPSSFDI

SEQ ID NO: 115 - DNA, 1116 bp, Homo Sapiens
atggagaccgacaccctgctgctgtgggtgctgctgctgtgggtgcccggatccaccggctctgaggtgcagctggaggagactggaggagacttgatccagccgggggggtccctgagactctcctgtacagcctctgggtttaacgtcagtagaatctacatgagctgggtccgccaggctccagggaaggggctggagtgggtctcagtgatttatagcggtggaagtatatattacgcagattccgtgaggggccgatttaccatctccagagacagttccacgaacacggtgtttcttcaaatgaacagcctgagagccgaggactcggccgtgtattactgtgcgagagccgtcccaagtgcccctagttcttttgatatctggggccaagggacaatggtcaccgtctcttcagagcccaaatcttgtgacaaaactcacacatgcccaccgtgcccagcacctgaactcctggggggaccggacgtcttcctcttccccccaaaacccaaggacaccctcatgatctcccggacccctgaggtcacatgcgtggtggtggacgtgagccacgaagaccctgaggtcaagttcaactggtacgtggacggcgtggaggtgcataatgccaagacaaagccgcgggaggagcagtacaacagcacgtaccgggtggtcagcgtcctcaccgtcctgcaccaggactggctgaatggcaaggagtacaagtgcaaggtctccaacaaagccctcccagcccccgaggagaaaaccatctccaaagccaaagggcagccccgagaaccacaggtgtacaccctgcccccatcccgggaggagatgaccaagaaccaggtcagcctgacctgcctggtcaaaggcttctatcccagcgacatcgccgtggagtgggagagcaatgggcagccggagaacaactacaagaccacgcctcccgtgctggactccgacggctccttcttcctctacagcaagctcaccgtggacaagagcaggtggcagcaggggaacgtcttctcatgctccgtgatgcatgaggctctgcacaaccactacacgcagaagagcctctccctgtctccgggtaaa

SEQ ID NO: 116 - protein, 372 aa, Homo Sapiens
METDTLLLWVLLLWVPGSTGSEVQLEETGGDLIQPGGSLRLSCTASGFNVSRIYMSWVRQAPGKGLEWVSVIYSGGSIYYADSVRGRFTISRDSSTNTVFLQMNSLRAEDSAVYYCARAVPSAPSSFDIWGQGTMVTVSSEPKSCDKTHTCPPCPAPELLGGPDVFLFPPKPKDTLMISRTPEVTCVVVDVSHEDPEVKFNWYVDGVEVHNAKTKPREEQYNSTYRVVSVLTVLHQDWLNGKEYKCKVSNKALPAPEEKTISKAKGQPREPQVYTLPPSREEMTKNQVSLTCLVKGFYPSDIAVEWESNGQPENNYKTTPPVLDSDGSFFLYSKLTVDKSRWQQGNVFSCSVMHEALHNHYTQKSLSLSPGK

SEQ ID NO: 117 - protein, 119 aa, Homo Sapiens; identical to SEQ ID NO: 15

SEQ ID NO: 118 - protein, 10 aa, Homo Sapiens
GFNVSRIYMS

SEQ ID NO: 119 - protein, 16 aa, Homo Sapiens
VIYSGGSIYYADSVRG

SEQ ID NO: 120 - protein, 11 aa, Homo Sapiens
AVPSAPSSFDI

SEQ ID NO: 121 - DNA, 1116 bp, Homo Sapiens
atggagaccgacaccctgctgctgtgggtgctgctgctgtgggtgcccggatccaccggctctgaggtgcagctggtggagactggaggagggctgatccagccgggggggtccctgagactctcctgtgcagtctctgggttcaccgtcagaaacaactacatgagctgggcccgccaggttccagggaagggactggagtgggtctcagttatttatagcggtgggagtataacctacgcagactccgtgaagggccgattcatcatctccagagacaattccaacaacacgctatatcttcaaatgaacggtctgagagccgaggacacggccgtatattactgtgcgagagccgtcccacatgccccaagtgcttttgacatctggggccaggggacaatggtcaccgtctcttcagagcccaaatcttgtgacaaaactcacacatgcccaccgtgcccagcacctgaactcctggggggaccggacgtcttcctcttccccccaaaacccaaggacaccctcatgatctcccggacccctgaggtcacatgcgtggtggtggacgtgagccacgaagaccctgaggtcaagttcaactggtacgtggacggcgtggaggtgcataatgccaagacaaagccgcgggaggagcagtacaacagcacgtaccgggtggtcagcgtcctcaccgtcctgcaccaggactggctgaatggcaaggagtacaagtgcaaggtctccaacaaagccctcccagcccccgaggagaaaaccatctccaaagccaaagggcagccccgagaaccacaggtgtacaccctgcccccatcccgggaggagatgaccaagaaccaggtcagcctgacctgcctggtcaaaggcttctatcccagcgacatcgccgtggagtgggagagcaatgggcagccggagaacaactacaagaccacgcctcccgtgctggactccgacggctccttcttcctctacagcaagctcaccgtggacaagagcaggtggcagcaggggaacgtcttctcatgctccgtgatgcatgaggctctgcacaaccactacacgcagaagagcctctccctgtctccgggtaaa

SEQ ID NO: 122 - protein, 372 aa, Homo Sapiens
METDTLLLWVLLLWVPGSTGSEVQLVETGGGLIQPGGSLRLSCAVSGFTVRNNYMSWARQVPGKGLEWVSVIYSGGSITYADSVKGRFIISRDNSNNTLYLQMNGLRAEDTAVYYCARAVPHAPSAFDIWGQGTMVTVSSEPKSCDKTHTCPPCPAPELLGGPDVFLFPPKPKDTLMISRTPEVTCVVVDVSHEDPEVKFNWYVDGVEVHNAKTKPREEQYNSTYRVVSVLTVLHQDWLNGKEYKCKVSNKALPAPEEKTISKAKGQPREPQVYTLPPSREEMTKNQVSLTCLVKGFYPSDIAVEWESNGQPENNYKTTPPVLDSDGSFFLYSKLTVDKSRWQQGNVFSCSVMHEALHNHYTQKSLSLSPGK

SEQ ID NO: 123 - protein, 119 aa, Homo Sapiens; identical to SEQ ID NO: 27

SEQ ID NO: 124 - protein, 10 aa, Homo Sapiens
GFTVRNNYMS

SEQ ID NO: 125 - protein, 16 aa, Homo Sapiens
VIYSGGSITYADSVKG

SEQ ID NO: 126 - protein, 11 aa, Homo Sapiens
AVPHAPSAFDI

SEQ ID NO: 127 - DNA, 1116 bp, Homo Sapiens
atggagaccgacaccctgctgctgtgggtgctgctgctgtgggtgcccggatccaccggctctgaggtgcagctggtggagactggaggaggcttgatccagcctggggggtccctgagactctcctgtgcagcctctgggttcaccgtcagtagcaactacatgagctgggtccgccaggctccagggaaggggctggagtgggtctcagttatttatagcggtggtagcacatactacgcagactccgtgaagggccgattcaccatctccagagacaattccaagaacacgctgtatcttcaaatgagcaacctgaccgccgaggacacggccgtgtattactgtgcgagagccgttccccactcccccagtgcttttgataggtggggccagggaaccctggtcaccgtctcttcagagcccaaatcttgtgacaaaactcacacatgcccaccgtgcccagcacctgaactcctggggggaccggacgtcttcctcttccccccaaaacccaaggacaccctcatgatctcccggacccctgaggtcacatgcgtggtggtggacgtgagccacgaagaccctgaggtcaagttcaactggtacgtggacggcgtggaggtgcataatgccaagacaaagccgcgggaggagcagtacaacagcacgtaccgggtggtcagcgtcctcaccgtcctgcaccaggactggctgaatggcaaggagtacaagtgcaaggtctccaacaaagccctcccagcccccgaggagaaaaccatctccaaagccaaagggcagccccgagaaccacaggtgtacaccctgcccccatcccgggaggagatgaccaagaaccaggtcagcctgacctgcctggtcaaaggcttctatcccagcgacatcgccgtggagtgggagagcaatgggcagccggagaacaactacaagaccacgcctcccgtgctggactccgacggctccttcttcctctacagcaagctcaccgtggacaagagcaggtggcagcaggggaacgtcttctcatgctccgtgatgcatgaggctctgcacaaccactacacgcagaagagcctctccctgtctccgggtaaa

SEQ ID NO: 128 - protein, 372 aa, Homo Sapiens
METDTLLLWVLLLWVPGSTGSEVQLVETGGGLIQPGGSLRLSCAASGFTVSSNYMSWVRQAPGKGLEWVSVIYSGGSTYYADSVKGRFTISRDNSKNTLYLQMSNLTAEDTAVYYCARAVPHSPSAFDRWGQGTLVTVSSEPKSCDKTHTCPPCPAPELLGGPDVFLFPPKPKDTLMISRTPEVTCVVVDVSHEDPEVKFNWYVDGVEVHNAKTKPREEQYNSTYRVVSVLTVLHQDWLNGKEYKCKVSNKALPAPEEKTISKAKGQPREPQVYTLPPSREEMTKNQVSLTCLVKGFYPSDIAVEWESNGQPENNYKTTPPVLDSDGSFFLYSKLTVDKSRWQQGNVFSCSVMHEALHNHYTQKSLSLSPGK

SEQ ID NO: 129 - protein, 119 aa, Homo Sapiens; identical to SEQ ID NO: 39

SEQ ID NO: 130 - protein, 10 aa, Homo Sapiens
GFTVSSNYMS

SEQ ID NO: 131 - protein, 16 aa, Homo Sapiens
VIYSGGSTYYADSVKG

SEQ ID NO: 132 - protein, 11 aa, Homo Sapiens
AVPHSPSAFDR

SEQ ID NO: 133 - DNA, 1116 bp, Homo Sapiens
atggagaccgacaccctgctgctgtgggtgctgctgctgtgggtgcccggatccaccggctctgaggtgcagctggaggagactggaggagacttgatccagccgggggggtccctgagactctcctgtacagcctctgggtttaacgtcagtagaatctacatgagctgggtccgccaggctccagggaaggggctggagtgggtctcagtgatttatagcggtggaagtatatattacgcagattccgtgaggggccgatttaccatctccagagacagttccacgaacacggtgtatcttcaaatgaacagcctgagagccgaggactcggccgtgtattactgtgcgagagccgtcccacatgcccctagtaattttgataaatggggccaagggacaagggtcaccgtctcttcagagcccaaatcttgtgacaaaactcacacatgcccaccgtgcccagcacctgaactcctggggggaccggacgtcttcctcttccccccaaaacccaaggacaccctcatgatctcccggacccctgaggtcacatgcgtggtggtggacgtgagccacgaagaccctgaggtcaagttcaactggtacgtggacggcgtggaggtgcataatgccaagacaaagccgcgggaggagcagtacaacagcacgtaccgggtggtcagcgtcctcaccgtcctgcaccaggactggctgaatggcaaggagtacaagtgcaaggtctccaacaaagccctcccagcccccgaggagaaaaccatctccaaagccaaagggcagccccgagaaccacaggtgtacaccctgcccccatcccgggaggagatgaccaagaaccaggtcagcctgacctgcctggtcaaaggcttctatcccagcgacatcgccgtggagtgggagagcaatgggcagccggagaacaactacaagaccacgcctcccgtgctggactccgacggctccttcttcctctacagcaagctcaccgtggacaagagcaggtggcagcaggggaacgtcttctcatgctccgtgatgcatgaggctctgcacaaccactacacgcagaagagcctctccctgtctccgggtaaa

SEQ ID NO: 134 - protein, 372 aa, Homo Sapiens
METDTLLLWVLLLWVPGSTGSEVQLEETGGDLIQPGGSLRLSCTASGFNVSRIYMSWVRQAPGKGLEWVSVIYSGGSIYYADSVRGRFTISRDSSTNTVYLQMNSLRAEDSAVYYCARAVPHAPSNFDKWGQGTRVTVSSEPKSCDKTHTCPPCPAPELLGGPDVFLFPPKPKDTLMISRTPEVTCVVVDVSHEDPEVKFNWYVDGVEVHNAKTKPREEQYNSTYRVVSVLTVLHQDWLNGKEYKCKVSNKALPAPEEKTISKAKGQPREPQVYTLPPSREEMTKNQVSLTCLVKGFYPSDIAVEWESNGQPENNYKTTPPVLDSDGSFFLYSKLTVDKSRWQQGNVFSCSVMHEALHNHYTQKSLSLSPGK

SEQ ID NO: 135 - protein, 119 aa, Homo Sapiens; identical to SEQ ID NO: 45

SEQ ID NO: 136 - protein, 10 aa, Homo Sapiens
GFNVSRIYMS

SEQ ID NO: 137 - protein, 16 aa, Homo Sapiens
VIYSGGSIYYADSVRG

SEQ ID NO: 138 - protein, 11 aa, Homo Sapiens
AVPHAPSNFDK

SEQ ID NO: 139 - DNA, 1116 bp, Homo Sapiens
atggagaccgacaccctgctgctgtgggtgctgctgctgtgggtgcccggatccaccggctctgaggtgcagctggcggagactggaggaggcttgatccagcctggggggtccctgagactctcctgtgcagtctctgggttcaatgtcagtaagaattacatgagctgggtccgccaggttccagggaaggggctggagtgggtcgcagttgtttatagcggtggtagcaaaacctacgcagactccgtgaagggccgattcatcctctccagagacaattccgacaacacactgtatcttcaaatgaacaacctgagagccgaggacacggccgtgtattactgtgcgagagccgttcctcattcccccagttcttttgatatctggggccaagggacaatggtcaccgtctcttcagagcccaaatcttgtgacaaaactcacacatgcccaccgtgcccagcacctgaactcctggggggaccggacgtcttcctcttccccccaaaacccaaggacaccctcatgatctcccggacccctgaggtcacatgcgtggtggtggacgtgagccacgaagaccctgaggtcaagttcaactggtacgtggacggcgtggaggtgcataatgccaagacaaagccgcgggaggagcagtacaacagcacgtaccgggtggtcagcgtcctcaccgtcctgcaccaggactggctgaatggcaaggagtacaagtgcaaggtctccaacaaagccctcccagcccccgaggagaaaaccatctccaaagccaaagggcagccccgagaaccacaggtgtacaccctgcccccatcccgggaggagatgaccaagaaccaggtcagcctgacctgcctggtcaaaggcttctatcccagcgacatcgccgtggagtgggagagcaatgggcagccggagaacaactacaagaccacgcctcccgtgctggactccgacggctccttcttcctctacagcaagctcaccgtggacaagagcaggtggcagcaggggaacgtcttctcatgctccgtgatgcatgaggctctgcacaaccactacacgcagaagagcctctccctgtctccgggtaaa

SEQ ID NO: 140 - protein, 372 aa, Homo Sapiens
METDTLLLWVLLLWVPGSTGSEVQLAETGGGLIQPGGSLRLSCAVSGFNVSKNYMSWVRQVPGKGLEWVAVVYSGGSKTYADSVKGRFILSRDNSDNTLYLQMNNLRAEDTAVYYCARAVPHSPSSFDIWGQGTMVTVSSEPKSCDKTHTCPPCPAPELLGGPDVFLFPPKPKDTLMISRTPEVTCVVVDVSHEDPEVKFNWYVDGVEVHNAKTKPREEQYNSTYRVVSVLTVLHQDWLNGKEYKCKVSNKALPAPEEKTISKAKGQPREPQVYTLPPSREEMTKNQVSLTCLVKGFYPSDIAVEWESNGQPENNYKTTPPVLDSDGSFFLYSKLTVDKSRWQQGNVFSCSVMHEALHNHYTQKSLSLSPGK

SEQ ID NO: 141 - protein, 119 aa, Homo Sapiens; identical to SEQ ID NO: 9

SEQ ID NO: 142 - protein, 10 aa, Homo Sapiens
GFNVSKNYMS

SEQ ID NO: 143 - protein, 16 aa, Homo Sapiens
VVYSGGSKTYADSVKG

SEQ ID NO: 144 - protein, 11 aa, Homo Sapiens
AVPHSPSSFDI

SEQ ID NO: 145 - DNA, 1116 bp, Homo Sapiens
atggagaccgacaccctgctgctgtgggtgctgctgctgtgggtgcccggatccaccggctctgaggtgcagctggcggagactggaggaggcttgatccagcctggggggtccctgagactctcctgtgcagtctctgggttcaccgtcagtaagaattacatgagctgggtccgccaggttccagggaaggggctggagtgggtcgcagttgtttatagcggtggtagcaaaacctacgcagactccgtgaagggccgattcatcctctccagagacaattccgacaacacactgtatcttcaaatgaacaacctgagagccgaggacacggccgtgtattactgtgcgagagccgttcctcattcccccagttcttttgatatctggggccaagggacaatggtcaccgtctcttcagagcccaaatcttgtgacaaaactcacacatgcccaccgtgcccagcacctgaactcctggggggaccggacgtcttcctcttccccccaaaacccaaggacaccctcatgatctcccggacccctgaggtcacatgcgtggtggtggacgtgagccacgaagaccctgaggtcaagttcaactggtacgtggacggcgtggaggtgcataatgccaagacaaagccgcgggaggagcagtacaacagcacgtaccgggtggtcagcgtcctcaccgtcctgcaccaggactggctgaatggcaaggagtacaagtgcaaggtctccaacaaagccctcccagcccccgaggagaaaaccatctccaaagccaaagggcagccccgagaaccacaggtgtacaccctgcccccatcccgggaggagatgaccaagaaccaggtcagcctgacctgcctggtcaaaggcttctatcccagcgacatcgccgtggagtgggagagcaatgggcagccggagaacaactacaagaccacgcctcccgtgctggactccgacggctccttcttcctctacagcaagctcaccgtggacaagagcaggtggcagcaggggaacgtcttctcatgctccgtgatgcatgaggctctgcacaaccactacacgcagaagagcctctccctgtctccgggtaaa

SEQ ID NO: 146 - protein, 372 aa, Homo Sapiens
METDTLLLWVLLLWVPGSTGSEVQLAETGGGLIQPGGSLRLSCAVSGFTVSKNYMSWVRQVPGKGLEWVAVVYSGGSKTYADSVKGRFILSRDNSDNTLYLQMNNLRAEDTAVYYCARAVPHSPSSFDIWGQGTMVTVSSEPKSCDKTHTCPPCPAPELLGGPDVFLFPPKPKDTLMISRTPEVTCVVVDVSHEDPEVKFNWYVDGVEVHNAKTKPREEQYNSTYRVVSVLTVLHQDWLNGKEYKCKVSNKALPAPEEKTISKAKGQPREPQVYTLPPSREEMTKNQVSLTCLVKGFYPSDIAVEWESNGQPENNYKTTPPVLDSDGSFFLYSKLTVDKSRWQQGNVFSCSVMHEALHNHYTQKSLSLSPGK

SEQ ID NO: 147 - protein, 119 aa, Homo Sapiens; identical to SEQ ID NO: 105

SEQ ID NO: 148 - protein, 10 aa, Homo Sapiens
GFTVSKNYMS

SEQ ID NO: 149 - protein, 16 aa, Homo Sapiens
VVYSGGSKTYADSVKG

SEQ ID NO: 150 - protein, 11 aa, Homo Sapiens
AVPHSPSSFDI

SEQ ID NO: 151 - DNA, 1116 bp, Homo Sapiens
atggagaccgacaccctgctgctgtgggtgctgctgctgtgggtgcccggatccaccggctctgaggtgcagctggtggagagcggaggaggcttgatccagcctggggggtccctgagactctcctgtgcagtctctgggttcaccgtcagtaagaattacatgagctgggtccgccaggccccagggaaggggctggagtgggtcagcgttgtttatagcggtggtagcaaaacctacgcagactccgtgaagggccgattcaccatctccagagacaattccaagaacacactgtatcttcaaatgaacagcctgagagccgaggacacggccgtgtattactgtgcgagagccgttcctcattcccccagttcttttgatatctggggccaagggacaatggtcaccgtctcttcagagcccaaatcttgtgacaaaactcacacatgcccaccgtgcccagcacctgaactcctggggggaccggacgtcttcctcttccccccaaaacccaaggacaccctcatgatctcccggacccctgaggtcacatgcgtggtggtggacgtgagccacgaagaccctgaggtcaagttcaactggtacgtggacggcgtggaggtgcataatgccaagacaaagccgcgggaggagcagtacaacagcacgtaccgggtggtcagcgtcctcaccgtcctgcaccaggactggctgaatggcaaggagtacaagtgcaaggtctccaacaaagccctcccagcccccgaggagaaaaccatctccaaagccaaagggcagccccgagaaccacaggtgtacaccctgcccccatcccgggaggagatgaccaagaaccaggtcagcctgacctgcctggtcaaaggcttctatcccagcgacatcgccgtggagtgggagagcaatgggcagccggagaacaactacaagaccacgcctcccgtgctggactccgacggctccttcttcctctacagcaagctcaccgtggacaagagcaggtggcagcaggggaacgtcttctcatgctccgtgatgcatgaggctctgcacaaccactacacgcagaagagcctctccctgtctccgggtaaa

SEQ ID NO: 152 - protein, 372 aa, Homo Sapiens
METDTLLLWVLLLWVPGSTGSEVQLVESGGGLIQPGGSLRLSCAVSGFTVSKNYMSWVRQAPGKGLEWVSVVYSGGSKTYADSVKGRFTISRDNSKNTLYLQMNSLRAEDTAVYYCARAVPHSPSSFDIWGQGTMVTVSSEPKSCDKTHTCPPCPAPELLGGPDVFLFPPKPKDTLMISRTPEVTCVVVDVSHEDPEVKFNWYVDGVEVHNAKTKPREEQYNSTYRVVSVLTVLHQDWLNGKEYKCKVSNKALPAPEEKTISKAKGQPREPQVYTLPPSREEMTKNQVSLTCLVKGFYPSDIAVEWESNGQPENNYKTTPPVLDSDGSFFLYSKLTVDKSRWQQGNVFSCSVMHEALHNHYTQKSLSLSPGK

SEQ ID NO: 153 - protein, 119 aa, Homo Sapiens; identical to SEQ ID NO: 111

SEQ ID NO: 154 - protein, 10 aa, Homo Sapiens
GFTVSKNYMS

SEQ ID NO: 155 - protein, 16 aa, Homo Sapiens
VVYSGGSKTYADSVKG

SEQ ID NO: 156 - protein, 11 aa, Homo Sapiens
AVPHSPSSFDI

SEQ ID NO: 157 - DNA, 1116 bp, Homo Sapiens
atggagaccgacaccctgctgctgtgggtgctgctgctgtgggtgcccggatccaccggcgaggtgcagctggtggagtccgggggaggcttagttcagcctggggggtccctgagactctcctgtgcagcctctggattcaccttcagtaactactggatgcactgggtccgccaagctccagggaaggggctggtgtgggtctcacgtattaatagtgatgggagtaacacaacctacgcggactccgtgaagggccgattcaccatctccagagacaacgccaagaacacgctgtatctgcaaatgaacagtctgagagccgaggacacggctgtgtattactgtgcaagatggttcggggagcactactacggaatggacgtctggggccaagggaccacggtcaccgtctcttcagagcccaaatcttgtgacaaaactcacacatgcccaccgtgcccagcacctgaactcctggggggaccgtcagtcttcctcttccccccaaaacccaaggacaccctcatgatctcccggacccctgaggtcacatgcgtggtggtggacgtgagccacgaagaccctgaggtcaagttcaactggtacgtggacggcgtggaggtgcataatgccaagacaaagccgcgggaggagcagtacaacagcacgtaccgggtggtcagcgtcctcaccgtcctgcaccaggactggctgaatggcaaggagtacaagtgcaaggtctccaacaaagccctcccagcccccatcgagaaaaccatctccaaagccaaagggcagccccgagaaccacaggtgtacaccctgcccccatcccgggaggagatgaccaagaaccaggtcagcctgacctgcctggtcaaaggcttctatcccagcgacatcgccgtggagtgggagagcaatgggcagccggagaacaactacaagaccacgcctcccgtgctggactccgacggctccttcttcctctacagcaagctcaccgtggacaagagcaggtggcagcaggggaacgtcttctcatgctccgtgatgcatgaggctctgcacaaccactacacgcagaagagcctctccctgtctccgggtaaa

SEQ ID NO: 158 - protein, 372 aa, Homo Sapiens
METDTLLLWVLLLWVPGSTGEVQLVESGGGLVQPGGSLRLSCAASGFTFSNYWMHWVRQAPGKGLVWVSRINSDGSNTTYADSVKGRFTISRDNAKNTLYLQMNSLRAEDTAVYYCARWFGEHYYGMDVWGQGTTVTVSSEPKSCDKTHTCPPCPAPELLGGPSVFLFPPKPKDTLMISRTPEVTCVVVDVSHEDPEVKFNWYVDGVEVHNAKTKPREEQYNSTYRVVSVLTVLHQDWLNGKEYKCKVSNKALPAPIEKTISKAKGQPREPQVYTLPPSREEMTKNQVSLTCLVKGFYPSDIAVEWESNGQPENNYKTTPPVLDSDGSFFLYSKLTVDKSRWQQGNVFSCSVMHEALHNHYTQKSLSLSPGK

SEQ ID NO: 159 - protein, 120 aa, Homo Sapiens; identical to SEQ ID NO: 21

SEQ ID NO: 160 - protein, 10 aa, Homo Sapiens
GFTFSNYWMH

SEQ ID NO: 161 - protein, 17 aa, Homo Sapiens
RINSDGSNTTYADSVKG

SEQ ID NO: 162 - protein, 11 aa, Homo Sapiens
WFGEHYYGMDV

SEQ ID NO: 163 - DNA, 1113 bp, Homo Sapiens
atggagaccgacaccctgctgctgtgggtgctgctgctgtgggtgcccggatccaccggcgaggtgcagctggtggagagcggaggaggcttgatccagccgggggggtccctgagactctcctgtgccgcctctgggtttaccgtcagtagaatctacatgagctgggtccgccaggctccagggaaggggctggagtgggtctcagtgatttatagcggtggaagtatatattacgcagattccgtgaagggccgatttaccatctccagagacagttccaagaacacggtgtaccttcaaatgaacagcctgagagccgaggacaccgccgtgtattactgtgcgagagccgtcccaagtgcccctagttcttttgatatctggggccaagggacaatggtcaccgtctcttcagagcccaaatcttgtgacaaaactcacacatgcccaccgtgcccagcacctgaactcctggggggaccgtcagtcttcctcttccccccaaaacccaaggacaccctcatgatctcccggacccctgaggtcacatgcgtggtggtggacgtgagccacgaagaccctgaggtcaagttcaactggtacgtggacggcgtggaggtgcataatgccaagacaaagccgcgggaggagcagtacaacagcacgtaccgggtggtcagcgtcctcaccgtcctgcaccaggactggctgaatggcaaggagtacaagtgcaaggtctccaacaaagccctcccagcccccatcgagaaaaccatctccaaagccaaagggcagccccgagaaccacaggtgtacaccctgcccccatcccgggaggagatgaccaagaaccaggtcagcctgacctgcctggtcaaaggcttctatcccagcgacatcgccgtggagtgggagagcaatgggcagccggagaacaactacaagaccacgcctcccgtgctggactccgacggctccttcttcctctacagcaagctcaccgtggacaagagcaggtggcagcaggggaacgtcttctcatgctccgtgatgcatgaggctctgcacaaccactacacgcagaagagcctctccctgtctccgggtaaa

SEQ ID NO: 164 - protein, 371 aa, Homo Sapiens
METDTLLLWVLLLWVPGSTGEVQLVESGGGLIQPGGSLRLSCAASGFTVSRIYMSWVRQAPGKGLEWVSVIYSGGSIYYADSVKGRFTISRDSSKNTVYLQMNSLRAEDTAVYYCARAVPSAPSSFDIWGQGTMVTVSSEPKSCDKTHTCPPCPAPELLGGPSVFLFPPKPKDTLMISRTPEVTCVVVDVSHEDPEVKFNWYVDGVEVHNAKTKPREEQYNSTYRVVSVLTVLHQDWLNGKEYKCKVSNKALPAPIEKTISKAKGQPREPQVYTLPPSREEMTKNQVSLTCLVKGFYPSDIAVEWESNGQPENNYKTTPPVLDSDGSFFLYSKLTVDKSRWQQGNVFSCSVMHEALHNHYTQKSLSLSPGK

SEQ ID NO: 165 - protein, 119 aa, Homo Sapiens; identical to SEQ ID NO: 63

SEQ ID NO: 166 - protein, 10 aa, Homo Sapiens
GFTVSRIYMS

SEQ ID NO: 167 - protein, 16 aa, Homo Sapiens
VIYSGGSIYYADSVKG

SEQ ID NO: 168 - protein, 11 aa, Homo Sapiens
AVPSAPSSFDI

SEQ ID NO: 169 - DNA, 1113 bp, Homo Sapiens
atggagaccgacaccctgctgctgtgggtgctgctgctgtgggtgcccggatccaccggcgaggtgcagctggtggagagcggaggaggcttgatccagcctggggggtccctgagactctcctgtgcagtctctgggttcaccgtcagtaagaattacatgagctgggtccgccaggccccagggaaggggctggagtgggtcagcgttgtttatagcggtggtagcaaaacctacgcagactccgtgaagggccgattcaccatctccagagacaattccaagaacacactgtatcttcaaatgaacagcctgagagccgaggacacggccgtgtattactgtgcgagagccgttcctcattcccccagttcttttgatatctggggccaagggacaatggtcaccgtctcttcagagcccaaatcttgtgacaaaactcacacatgcccaccgtgcccagcacctgaactcctggggggaccgtcagtcttcctcttccccccaaaacccaaggacaccctcatgatctcccggacccctgaggtcacatgcgtggtggtggacgtgagccacgaagaccctgaggtcaagttcaactggtacgtggacggcgtggaggtgcataatgccaagacaaagccgcgggaggagcagtacaacagcacgtaccgggtggtcagcgtcctcaccgtcctgcaccaggactggctgaatggcaaggagtacaagtgcaaggtctccaacaaagccctcccagcccccatcgagaaaaccatctccaaagccaaagggcagccccgagaaccacaggtgtacaccctgcccccatcccgggaggagatgaccaagaaccaggtcagcctgacctgcctggtcaaaggcttctatcccagcgacatcgccgtggagtgggagagcaatgggcagccggagaacaactacaagaccacgcctcccgtgctggactccgacggctccttcttcctctacagcaagctcaccgtggacaagagcaggtggcagcaggggaacgtcttctcatgctccgtgatgcatgaggctctgcacaaccactacacgcagaagagcctctccctgtctccgggtaaa

SEQ ID NO: 170 - protein, 371 aa, Homo Sapiens
METDTLLLWVLLLWVPGSTGEVQLVESGGGLIQPGGSLRLSCAVSGFTVSKNYMSWVRQAPGKGLEWVSVVYSGGSKTYADSVKGRFTISRDNSKNTLYLQMNSLRAEDTAVYYCARAVPHSPSSFDIWGQGTMVTVSSEPKSCDKTHTCPPCPAPELLGGPSVFLFPPKPKDTLMISRTPEVTCVVVDVSHEDPEVKFNWYVDGVEVHNAKTKPREEQYNSTYRVVSVLTVLHQDWLNGKEYKCKVSNKALPAPIEKTISKAKGQPREPQVYTLPPSREEMTKNQVSLTCLVKGFYPSDIAVEWESNGQPENNYKTTPPVLDSDGSFFLYSKLTVDKSRWQQGNVFSCSVMHEALHNHYTQKSLSLSPGK

SEQ ID NO: 171 - protein, 119 aa, Homo Sapiens; identical to SEQ ID NO: 111

SEQ ID NO: 172 - protein, 10 aa, Homo Sapiens
GFTVSKNYMS

SEQ ID NO: 173 - protein, 16 aa, Homo Sapiens
VVYSGGSKTYADSVKG

SEQ ID NO: 174 - protein, 11 aa, Homo Sapiens
AVPHSPSSFDI

SEQ ID NO: 175 - DNA, 1113 bp, Homo Sapiens
atggagaccgacaccctgctgctgtgggtgctgctgctgtgggtgcccggatccaccggcgaggtgcagctggtggagagcggaggaggcttgatccagccgggggggtccctgagactctcctgtgccgcctctgggtttaccgtcagtagaatctacatgagctgggtccgccaggctccagggaaggggctggagtgggtctcagtgatttatagcggtggaagtatatattacgcagattccgtgaagggccgatttaccatctccagagacagttccaagaacacggtgtaccttcaaatgaacagcctgagagccgaggacaccgccgtgtattactgtgcgagagccgtcccaagtgcccctagttcttttgatatctggggccaagggacaatggtcaccgtctcttcagagcccaaatcttgtgacaaaactcacacatgcccaccgtgcccagcacctgaactcctggggggaccggacgtcttcctcttccccccaaaacccaaggacaccctcatgatctcccggacccctgaggtcacatgcgtggtggtggacgtgagccacgaagaccctgaggtcaagttcaactggtacgtggacggcgtggaggtgcataatgccaagacaaagccgcgggaggagcagtacaacagcacgtaccgggtggtcagcgtcctcaccgtcctgcaccaggactggctgaatggcaaggagtacaagtgcaaggtctccaacaaagccctcccagcccccgaggagaaaaccatctccaaagccaaagggcagccccgagaaccacaggtgtacaccctgcccccatcccgggaggagatgaccaagaaccaggtcagcctgacctgcctggtcaaaggcttctatcccagcgacatcgccgtggagtgggagagcaatgggcagccggagaacaactacaagaccacgcctcccgtgctggactccgacggctccttcttcctctacagcaagctcaccgtggacaagagcaggtggcagcaggggaacgtcttctcatgctccgtgatgcatgaggctctgcacaaccactacacgcagaagagcctctccctgtctccgggtaaa

SEQ ID NO: 176 - protein, 371 aa, Homo Sapiens
METDTLLLWVLLLWVPGSTGEVQLVESGGGLIQPGGSLRLSCAASGFTVSRIYMSWVRQAPGKGLEWVSVIYSGGSIYYADSVKGRFTISRDSSKNTVYLQMNSLRAEDTAVYYCARAVPSAPSSFDIWGQGTMVTVSSEPKSCDKTHTCPPCPAPELLGGPDVFLFPPKPKDTLMISRTPEVTCVVVDVSHEDPEVKFNWYVDGVEVHNAKTKPREEQYNSTYRVVSVLTVLHQDWLNGKEYKCKVSNKALPAPEEKTISKAKGQPREPQVYTLPPSREEMTKNQVSLTCLVKGFYPSDIAVEWESNGQPENNYKTTPPVLDSDGSFFLYSKLTVDKSRWQQGNVFSCSVMHEALHNHYTQKSLSLSPGK

SEQ ID NO: 177 - protein, 119 aa, Homo Sapiens; identical to SEQ ID NO: 63

SEQ ID NO: 178 - protein, 10 aa, Homo Sapiens
GFTVSRIYMS

SEQ ID NO: 179 - protein, 16 aa, Homo Sapiens
VIYSGGSIYYADSVKG

SEQ ID NO: 180 - protein, 11 aa, Homo Sapiens
AVPSAPSSFDI

SEQ ID NO: 181 - DNA, 1113 bp, Homo Sapiens
atggagaccgacaccctgctgctgtgggtgctgctgctgtgggtgcccggatccaccggcgaggtgcagctggtggagagcggaggaggcttgatccagcctggggggtccctgagactctcctgtgcagtctctgggttcaccgtcagtaagaattacatgagctgggtccgccaggccccagggaaggggctggagtgggtcagcgttgtttatagcggtggtagcaaaacctacgcagactccgtgaagggccgattcaccatctccagagacaattccaagaacacactgtatcttcaaatgaacagcctgagagccgaggacacggccgtgtattactgtgcgagagccgttcctcattcccccagttcttttgatatctggggccaagggacaatggtcaccgtctcttcagagcccaaatcttgtgacaaaactcacacatgcccaccgtgcccagcacctgaactcctggggggaccggacgtcttcctcttccccccaaaacccaaggacaccctcatgatctcccggacccctgaggtcacatgcgtggtggtggacgtgagccacgaagaccctgaggtcaagttcaactggtacgtggacggcgtggaggtgcataatgccaagacaaagccgcgggaggagcagtacaacagcacgtaccgggtggtcagcgtcctcaccgtcctgcaccaggactggctgaatggcaaggagtacaagtgcaaggtctccaacaaagccctcccagcccccgaggagaaaaccatctccaaagccaaagggcagccccgagaaccacaggtgtacaccctgcccccatcccgggaggagatgaccaagaaccaggtcagcctgacctgcctggtcaaaggcttctatcccagcgacatcgccgtggagtgggagagcaatgggcagccggagaacaactacaagaccacgcctcccgtgctggactccgacggctccttcttcctctacagcaagctcaccgtggacaagagcaggtggcagcaggggaacgtcttctcatgctccgtgatgcatgaggctctgcacaaccactacacgcagaagagcctctccctgtctccgggtaaa

SEQ ID NO: 182 - protein, 371 aa, Homo Sapiens
METDTLLLWVLLLWVPGSTGEVQLVESGGGLIQPGGSLRLSCAVSGFTVSKNYMSWVRQAPGKGLEWVSVVYSGGSKTYADSVKGRFTISRDNSKNTLYLQMNSLRAEDTAVYYCARAVPHSPSSFDIWGQGTMVTVSSEPKSCDKTHTCPPCPAPELLGGPDVFLFPPKPKDTLMISRTPEVTCVVVDVSHEDPEVKFNWYVDGVEVHNAKTKPREEQYNSTYRVVSVLTVLHQDWLNGKEYKCKVSNKALPAPEEKTISKAKGQPREPQVYTLPPSREEMTKNQVSLTCLVKGFYPSDIAVEWESNGQPENNYKTTPPVLDSDGSFFLYSKLTVDKSRWQQGNVFSCSVMHEALHNHYTQKSLSLSPGK

SEQ ID NO: 183 - protein, 119 aa, Homo Sapiens; identical to SEQ ID NO: 111

SEQ ID NO: 184 - protein, 10 aa, Homo Sapiens
GFTVSKNYMS

SEQ ID NO: 185 - protein, 16 aa, Homo Sapiens
VVYSGGSKTYADSVKG

SEQ ID NO: 186 - protein, 11 aa, Homo Sapiens
AVPHSPSSFDI

SEQ ID NO: 187 - DNA, 1116 bp, Homo Sapiens
atggagaccgacaccctgctgctgtgggtgctgctgctgtgggtgcccggatccaccggcgaggtgcagctggtggagtccgggggaggcttagttcagcctggggggtccctgagactctcctgtgcagcctctggattcaccttcagtaactactggatgcactgggtccgccaagctccagggaaggggctggtgtgggtctcacgtattaatagtgatgggagtaacacaacctacgcggactccgtgaagggccgattcaccatctccagagacaacgccaagaacacgctgtatctgcaaatgaacagtctgagagccgaggacacggctgtgtattactgtgcaagatggttcggggagcactactacggaatggacgtctggggccaagggaccacggtcaccgtctcttcagagcccaaatcttgtgacaaaactcacacatgcccaccgtgcccagcacctgaactcctggggggaccggacgtcttcctcttccccccaaaacccaaggacaccctcatgatctcccggacccctgaggtcacatgcgtggtggtggacgtgagccacgaagaccctgaggtcaagttcaactggtacgtggacggcgtggaggtgcataatgccaagacaaagccgcgggaggagcagtacaacagcacgtaccgggtggtcagcgtcctcaccgtcctgcaccaggactggctgaatggcaaggagtacaagtgcaaggtctccaacaaagccctcccagcccccgaggagaaaaccatctccaaagccaaagggcagccccgagaaccacaggtgtacaccctgcccccatcccgggaggagatgaccaagaaccaggtcagcctgacctgcctggtcaaaggcttctatcccagcgacatcgccgtggagtgggagagcaatgggcagccggagaacaactacaagaccacgcctcccgtgctggactccgacggctccttcttcctctacagcaagctcaccgtggacaagagcaggtggcagcaggggaacgtcttctcatgctccgtgatgcatgaggctctgcacaaccactacacgcagaagagcctctccctgtctccgggtaaa

SEQ ID NO: 188 - protein, 372 aa, Homo Sapiens
METDTLLLWVLLLWVPGSTGEVQLVESGGGLVQPGGSLRLSCAASGFTFSNYWMHWVRQAPGKGLVWVSRINSDGSNTTYADSVKGRFTISRDNAKNTLYLQMNSLRAEDTAVYYCARWFGEHYYGMDVWGQGTTVTVSSEPKSCDKTHTCPPCPAPELLGGPDVFLFPPKPKDTLMISRTPEVTCVVVDVSHEDPEVKFNWYVDGVEVHNAKTKPREEQYNSTYRVVSVLTVLHQDWLNGKEYKCKVSNKALPAPEEKTISKAKGQPREPQVYTLPPSREEMTKNQVSLTCLVKGFYPSDIAVEWESNGQPENNYKTTPPVLDSDGSFFLYSKLTVDKSRWQQGNVFSCSVMHEALHNHYTQKSLSLSPGK

SEQ ID NO: 189 - protein, 120 aa, Homo Sapiens; identical to SEQ ID NO: 21

SEQ ID NO: 190 - protein, 10 aa, Homo Sapiens
GFTFSNYWMH

SEQ ID NO: 191 - protein, 17 aa, Homo Sapiens
RINSDGSNTTYADSVKG

SEQ ID NO: 192 - protein, 11 aa, Homo Sapiens
WFGEHYYGMDV

SEQ ID NO: 193 - DNA, 23 bp, Artificial sequence
  Primer
gtgtccagtgtgaggtgcagctg

SEQ ID NO: 194 - DNA, 23 bp, Artificial sequence
  Primer
gtgtccagtgtcaggtgcagctg

SEQ ID NO: 195 - DNA, 24 bp, Artificial sequence
  Primer
ggcttacaaccacaatccctgggc

SEQ ID NO: 196 - DNA, 672 bp, Homo Sapiens
atggcttgccttggatttcagcggcacaaggctcagctgaacctggctaccaggacctggccctgcactctcctgttttttcttctcttcatccctgtcttctgcaaagcaatgcacgtggcccagcctgctgtggtactggccagcagccgaggcatcgccagctttgtgtgtgagtatgcatctccaggcaaagccactgaggtccgggtgacagtgcttcggcaggctgacagccaggtgactgaagtctgtgcggcaacctacatgatggggaatgagttgaccttcctagatgattccatctgcacgggcacctccagtggaaatcaagtgaacctcactatccaaggactgagggccatggacacgggactctacatctgcaaggtggagctcatgtacccaccgccatactacctgggcataggcaacggaacccagatttatgtaattgatccagaaccgtgcccagattctgacttcctcctctggatccttgcagcagttagttcggggttgtttttttatagctttctcctcacagctgtttctttgagcaaaatgctaaagaaaagaagccctcttacaacaggggtctatgtgaaaatgcccccaacagagccagaatgtgaaaagcaatttcagccttattttattcccatcaattga

SEQ ID NO: 197 - protein, 223 aa, Homo Sapiens
MACLGFQRHKAQLNLATRTWPCTLLFFLLFIPVFCKAMHVAQPAVVLASSRGIASFVCEYASPGKATEVRVTVLRQADSQVTEVCAATYMMGNELTFLDDSICTGTSSGNQVNLTIQGLRAMDTGLYICKVELMYPPPYYLGIGNGTQIYVIDPEPCPDSDFLLWILAAVSSGLFFYSFLLTAVSLSKMLKKRSPLTTGVYVKMPPTEPECEKQFQPYFIPIN

SEQ ID NO: 198 - DNA, 672 bp, Macaca mulatta
atggcttgccttggatttcagcggcacaaggctcggctcaacctggctaccaggacccggccctacactctcctgttttctcttctcttcatccctgtcttctccaaagcaatgcacgtggcccagcctgctgtggtgctggccaacagccgagggatcgccagctttgtgtgtgagtatgcatctccaggcaaagccactgaggtccgggtgacagtgcttcggcaggccgacagccaggtgactgaagtctgtgcggcaacatacatgatggggaatgagttgaccttcctagatgattccatctgcacgggcacctccagtggaaatcaagtgaacctcactatccaaggactgagggctatggacacaggactctacatctgcaaggtggagctcatgtacccaccaccatactacatgggcataggcaatggaacccagatttatgtaattgatccagaaccgtgcccagattctgacttcctcctctggatccttgcagcagttagttcggggttgtttttttatagctttctcctcacagctgtttctttgagcaaaatgctaaagaaaagaagccctctcacaacaggggtctatgtgaaaatgcccccaacagagccagaatgtgaaaagcaatttcagccttattttattcccatcaattga

SEQ ID NO: 199 - protein, 448 aa, Artificial sequence
  heavy chain of Ipilimumab analogue
QVQLVESGGGVVQPGRSLRLSCAASGFTFSSYTMHWVRQAPGKGLEWVTFISYDGNNKYYADSVKGRFTISRDNSKNTLYLQMNSLRAEDTAIYYCARTGWLGPFDYWGQGTLVTVSSASTKGPSVFPLAPSSKSTSGGTAALGCLVKDYFPEPVTVSWNSGALTSGVHTFPAVLQSSGLYSLSSVVTVPSSSLGTQTYICNVNHKPSNTKVDKKVEPKSCDKTHTCPPCPAPELLGGPSVFLFPPKPKDTLMISRTPEVTCVVVDVSHEDPEVKFNWYVDGVEVHNAKTKPREEQYNSTYRVVSVLTVLHQDWLNGKEYKCKVSNKALPAPIEKTISKAKGQPREPQVYTLPPSREEMTKNQVSLTCLVKGFYPSDIAVEWESNGQPENNYKTTPPVLDSDGSFFLYSKLTVDKSRWQQGNVFSCSVMHEALHNHYTQKSLSLSPGK

SEQ ID NO: 200 - protein, 215 aa, Artificial sequence
  light chain of Ipilimumab analogue
EIVLTQSPGTLSLSPGERATLSCRASQSVGSSYLAWYQQKPGQAPRLLIYGAFSRATGIPDRFSGSGSGTDFTLTISRLEPEDFAVYYCQQYGSSPWTFGQGTKVEIKRTVAAPSVFIFPPSDEQLKSGTASVVCLLNNFYPREAKVQWKVDNALQSGNSQESVTEQDSKDSTYSLSSTLTLSKADYEKHKVYACEVTHQGLSSPVTKSFNRGEC